European Patent Application EP 4 245 373 A2, published September 20, 2023. Title: ANTIBODIES AGAINST SARS-COV-2 AND METHODS OF USING THE SAME. Applicant: Vir Biotechnology, Inc. Application EP. The sequence listing filed with the application follows.

SEQUENCE LISTING (267 sequences)

SEQ ID NO: 1 - protein, 123 aa, synthetic construct
  REGION 1..123: note = Synthetic sequence SARS-CoV-2 S300-v1 mAb VH
QVQLVQSGAEVKKPGASVKVSCKASGYTFTDYYIHWVRQAPGQGPEWLGWVNGYSGATRYAQKYQGRVTMTRDTSISTAYMQLSRLRPDDTAVYYCARDRPSHEWAMYFFDNWGQGTLVTVSS

SEQ ID NO: 2 - protein, 8 aa, synthetic construct
  REGION 1..8: note = Synthetic sequence SARS-CoV-2 S300-v1 mAb CDRH1
GYTFTDYY

SEQ ID NO: 3 - protein, 8 aa, synthetic construct
  REGION 1..8: note = Synthetic sequence SARS-CoV-2 S300-v1 mAb CDRH2
VNGYSGAT

SEQ ID NO: 4 - protein, 16 aa, synthetic construct
  REGION 1..16: note = Synthetic sequence SARS-CoV-2 S300-v1 mAb CDRH3
ARDRPSHEWAMYFFDN

SEQ ID NO: 5 - protein, 109 aa, synthetic construct
  REGION 1..109: note = Synthetic sequence SARS-CoV-2 S300-v1 mAb VL (VK)
QIVLTQSPGTLSLSPGERATLSCRASQSVPSSCLAWYQQKPGQAPRLLIYGASGRATGIPDRFSGSGSGTDFTLTIRRLEPEDFAVYYCQQYGSSPPLTFGGGTKVEIK

SEQ ID NO: 6 - protein, 7 aa, synthetic construct
  REGION 1..7: note = Synthetic sequence SARS-CoV-2 S300-v1 mAb CDRL1
QSVPSSC

SEQ ID NO: 7 - skipped

SEQ ID NO: 8 - protein, 10 aa, synthetic construct
  REGION 1..10: note = Synthetic sequence SARS-CoV-2 S300-v1 mAb CDRL3
QQYGSSPPLT

SEQ ID NO: 9 - protein, 123 aa, synthetic construct
  REGION 1..123: note = Synthetic sequence SARS-CoV-2 S300-v1.1 mAb VH
QVQLVQSGAEVKKPGASVKVSCKASGYTFTDYYIHWVRQAPGQGPEWLGWVQGYSGATRYAQKYQGRVTMTRDTSISTAYMQLSRLRPDDTAVYYCARDRPSHEWAMYFFDNWGQGTLVTVSS

SEQ ID NO: 10 - protein, 123 aa, synthetic construct
  REGION 1..123: note = Synthetic sequence SARS-CoV-2 S300-v1.2 mAb VH
QVQLVQSGAEVKKPGASVKVSCKASGYTFTDYYIHWVRQAPGQGPEWLGWVNAYSGATRYAQKYQGRVTMTRDTSISTAYMQLSRLRPDDTAVYYCARDRPSHEWAMYFFDNWGQGTLVTVSS

SEQ ID NO: 11 - protein, 123 aa, synthetic construct
  REGION 1..123: note = Synthetic sequence SARS-CoV-2 S300-v1.3 mAb VH
QVQLVQSGAEVKKPGASVKVSCKASGYTFTDYYIHWVRQAPGQGPEWLGWVNSYSGATRYAQKYQGRVTMTRDTSISTAYMQLSRLRPDDTAVYYCARDRPSHEWAMYFFDNWGQGTLVTVSS

SEQ ID NO: 12 - protein, 123 aa, synthetic construct
  REGION 1..123: note = Synthetic sequence SARS-CoV-2 S300-v1.4 mAb VH
QVQLVQSGAEVKKPGASVKVSCKASGYTFTDYYIHWVRQAPGQGPEWLGWVNPYSGATRYAQKYQGRVTMTRDTSISTAYMQLSRLRPDDTAVYYCARDRPSHEWAMYFFDNWGQGTLVTVSS

SEQ ID NO: 13 - protein, 123 aa, synthetic construct
  REGION 1..123: note = Synthetic sequence SARS-CoV-2 S300-v1.5 mAb VH
QVQLVQSGAEVKKPGASVKVSCKASGYTFTDYYIHWVRQAPGQGPEWLGWVNQYSGATRYAQKYQGRVTMTRDTSISTAYMQLSRLRPDDTAVYYCARDRPSHEWAMYFFDNWGQGTLVTVSS

SEQ ID NO: 14 - protein, 123 aa, synthetic construct
  REGION 1..123: note = Synthetic sequence SARS-CoV-2 S300-v1.6 mAb VH
QVQLVQSGAEVKKPGASVKVSCKASGYTFTDYYIHWVRQAPGQGPEWLGWVLGYSGATRYAQKYQGRVTMTRDTSISTAYMQLSRLRPDDTAVYYCARDRPSHEWAMYFFDNWGQGTLVTVSS

SEQ ID NO: 15 - protein, 123 aa, synthetic construct
  REGION 1..123: note = Synthetic sequence SARS-CoV-2 S300-v1.7 mAb VH
QVQLVQSGAEVKKPGASVKVSCKASGYTFTDYYIHWVRQAPGQGPEWLGWVTGYSGATRYAQKYQGRVTMTRDTSISTAYMQLSRLRPDDTAVYYCARDRPSHEWAMYFFDNWGQGTLVTVSS

SEQ ID NO: 16 - protein, 8 aa, synthetic construct
  REGION 1..8: note = Synthetic sequence SARS-CoV-2 S300-v1.1 mAb CDRH2
VQGYSGAT

SEQ ID NO: 17 - protein, 8 aa, synthetic construct
  REGION 1..8: note = Synthetic sequence SARS-CoV-2 S300-v1.2 mAb CDRH2
VNAYSGAT

SEQ ID NO: 18 - protein, 8 aa, synthetic construct
  REGION 1..8: note = Synthetic sequence SARS-CoV-2 S300-v1.3 mAb CDRH2
VNSYSGAT

SEQ ID NO: 19 - protein, 8 aa, synthetic construct
  REGION 1..8: note = Synthetic sequence SARS-CoV-2 S300-v1.4 mAb CDRH2
VNPYSGAT

SEQ ID NO: 20 - protein, 8 aa, synthetic construct
  REGION 1..8: note = Synthetic sequence SARS-CoV-2 S300-v1.5 mAb CDRH2
VNQYSGAT

SEQ ID NO: 21 - protein, 8 aa, synthetic construct
  REGION 1..8: note = Synthetic sequence SARS-CoV-2 S300-v1.6 mAb CDRH2
VLGYSGAT

SEQ ID NO: 22 - protein, 8 aa, synthetic construct
  REGION 1..8: note = Synthetic sequence SARS-CoV-2 S300-v1.7 mAb CDRH2
VTGYSGAT

SEQ ID NO: 23 - protein, 123 aa, synthetic construct
  REGION 1..123: note = Synthetic sequence SARS-CoV-2 S300-v1.8 mAb VH
QVQLVQSGAEVKKPGASVKVSCKASGYTFTDYYIHWVRQAPGQGPEWLGWVNGYSGATRYAQKYQGRVTMTRDTSISTAYMQLSRLRPDDTAVYYCARDRPSHEFAMYFFDNWGQGTLVTVSS

SEQ ID NO: 24 - protein, 123 aa, synthetic construct
  REGION 1..123: note = Synthetic sequence SARS-CoV-2 S300-v1.9 mAb VH
QVQLVQSGAEVKKPGASVKVSCKASGYTFTDYYIHWVRQAPGQGPEWLGWVNGYSGATRYAQKYQGRVTMTRDTSISTAYMQLSRLRPDDTAVYYCARDRPSHEYAMYFFDNWGQGTLVTVSS

SEQ ID NO: 25 - protein, 16 aa, synthetic construct
  REGION 1..16: note = Synthetic sequence SARS-CoV-2 S300-v1.8 mAb CDRH3
ARDRPSHEFAMYFFDN

SEQ ID NO: 26 - protein, 16 aa, synthetic construct
  REGION 1..16: note = Synthetic sequence SARS-CoV-2 S300-v1.9 mAb CDRH3
ARDRPSHEYAMYFFDN

SEQ ID NO: 27 - protein, 123 aa, synthetic construct
  REGION 1..123: note = Synthetic sequence SARS-CoV-2 S300-v2 mAb VH
QVQLVQSGAEVKKPGASVKVSCKASGYTFTDYYIHWVRQAPGQGPEWLGFVNGYSGATRYAQKYQGRVTMTRDTSISTAYMQLSRLRPDDTAVYYCARDRPSHEWAMYFFDNWGQGTLVTVSS

SEQ ID NO: 28 - protein, 123 aa, synthetic construct
  REGION 1..123: note = Synthetic sequence SARS-CoV-2 S300-v2.1 mAb VH
QVQLVQSGAEVKKPGASVKVSCKASGYTFTDYYIHWVRQAPGQGPEWLGFVQGYSGATRYAQKYQGRVTMTRDTSISTAYMQLSRLRPDDTAVYYCARDRPSHEWAMYFFDNWGQGTLVTVSS

SEQ ID NO: 29 - protein, 123 aa, synthetic construct
  REGION 1..123: note = Synthetic sequence SARS-CoV-2 S300-v2.2 mAb VH
QVQLVQSGAEVKKPGASVKVSCKASGYTFTDYYIHWVRQAPGQGPEWLGFVNAYSGATRYAQKYQGRVTMTRDTSISTAYMQLSRLRPDDTAVYYCARDRPSHEWAMYFFDNWGQGTLVTVSS

SEQ ID NO: 30 - protein, 123 aa, synthetic construct
  REGION 1..123: note = Synthetic sequence SARS-CoV-2 S300-v2.3 mAb VH
QVQLVQSGAEVKKPGASVKVSCKASGYTFTDYYIHWVRQAPGQGPEWLGFVNSYSGATRYAQKYQGRVTMTRDTSISTAYMQLSRLRPDDTAVYYCARDRPSHEWAMYFFDNWGQGTLVTVSS

SEQ ID NO: 31 - protein, 123 aa, synthetic construct
  REGION 1..123: note = Synthetic sequence SARS-CoV-2 S300-v2.4 mAb VH
QVQLVQSGAEVKKPGASVKVSCKASGYTFTDYYIHWVRQAPGQGPEWLGFVNPYSGATRYAQKYQGRVTMTRDTSISTAYMQLSRLRPDDTAVYYCARDRPSHEWAMYFFDNWGQGTLVTVSS

SEQ ID NO: 32 - protein, 123 aa, synthetic construct
  REGION 1..123: note = Synthetic sequence SARS-CoV-2 S300-v2.5 mAb VH
QVQLVQSGAEVKKPGASVKVSCKASGYTFTDYYIHWVRQAPGQGPEWLGFVNQYSGATRYAQKYQGRVTMTRDTSISTAYMQLSRLRPDDTAVYYCARDRPSHEWAMYFFDNWGQGTLVTVSS

SEQ ID NO: 33 - protein, 123 aa, synthetic construct
  REGION 1..123: note = Synthetic sequence SARS-CoV-2 S300-v2.6 mAb VH
QVQLVQSGAEVKKPGASVKVSCKASGYTFTDYYIHWVRQAPGQGPEWLGFVLGYSGATRYAQKYQGRVTMTRDTSISTAYMQLSRLRPDDTAVYYCARDRPSHEWAMYFFDNWGQGTLVTVSS

SEQ ID NO: 34 - protein, 123 aa, synthetic construct
  REGION 1..123: note = Synthetic sequence SARS-CoV-2 S300-v2.7 mAb VH
QVQLVQSGAEVKKPGASVKVSCKASGYTFTDYYIHWVRQAPGQGPEWLGFVTGYSGATRYAQKYQGRVTMTRDTSISTAYMQLSRLRPDDTAVYYCARDRPSHEWAMYFFDNWGQGTLVTVSS

SEQ ID NO: 35 - protein, 123 aa, synthetic construct
  REGION 1..123: note = Synthetic sequence SARS-CoV-2 S300-v2.8 mAb VH
QVQLVQSGAEVKKPGASVKVSCKASGYTFTDYYIHWVRQAPGQGPEWLGFVNGYSGATRYAQKYQGRVTMTRDTSISTAYMQLSRLRPDDTAVYYCARDRPSHEFAMYFFDNWGQGTLVTVSS

SEQ ID NO: 36 - protein, 123 aa, synthetic construct
  REGION 1..123: note = Synthetic sequence SARS-CoV-2 S300-v2.9 mAb VH
QVQLVQSGAEVKKPGASVKVSCKASGYTFTDYYIHWVRQAPGQGPEWLGFVNGYSGATRYAQKYQGRVTMTRDTSISTAYMQLSRLRPDDTAVYYCARDRPSHEYAMYFFDNWGQGTLVTVSS

SEQ ID NO: 37 - protein, 123 aa, synthetic construct
  REGION 1..123: note = Synthetic sequence SARS-CoV-2 S300-v3 mAb VH
QVQLVQSGAEVKKPGASVKVSCKASGYTFTDYYIHWVRQAPGQGPEWLGYVNGYSGATRYAQKYQGRVTMTRDTSISTAYMQLSRLRPDDTAVYYCARDRPSHEWAMYFFDNWGQGTLVTVSS

SEQ ID NO: 38 - protein, 123 aa, synthetic construct
  REGION 1..123: note = Synthetic sequence SARS-CoV-2 S300-v3.1 mAb VH
QVQLVQSGAEVKKPGASVKVSCKASGYTFTDYYIHWVRQAPGQGPEWLGYVQGYSGATRYAQKYQGRVTMTRDTSISTAYMQLSRLRPDDTAVYYCARDRPSHEWAMYFFDNWGQGTLVTVSS

SEQ ID NO: 39 - protein, 123 aa, synthetic construct
  REGION 1..123: note = Synthetic sequence SARS-CoV-2 S300-v3.2 mAb VH
QVQLVQSGAEVKKPGASVKVSCKASGYTFTDYYIHWVRQAPGQGPEWLGYVNAYSGATRYAQKYQGRVTMTRDTSISTAYMQLSRLRPDDTAVYYCARDRPSHEWAMYFFDNWGQGTLVTVSS

SEQ ID NO: 40 - protein, 123 aa, synthetic construct
  REGION 1..123: note = Synthetic sequence SARS-CoV-2 S300-v3.3 mAb VH
QVQLVQSGAEVKKPGASVKVSCKASGYTFTDYYIHWVRQAPGQGPEWLGYVNSYSGATRYAQKYQGRVTMTRDTSISTAYMQLSRLRPDDTAVYYCARDRPSHEWAMYFFDNWGQGTLVTVSS

SEQ ID NO: 41 - protein, 123 aa, synthetic construct
  REGION 1..123: note = Synthetic sequence SARS-CoV-2 S300-v3.4 mAb VH
QVQLVQSGAEVKKPGASVKVSCKASGYTFTDYYIHWVRQAPGQGPEWLGYVNPYSGATRYAQKYQGRVTMTRDTSISTAYMQLSRLRPDDTAVYYCARDRPSHEWAMYFFDNWGQGTLVTVSS

SEQ ID NO: 42 - protein, 123 aa, synthetic construct
  REGION 1..123: note = Synthetic sequence SARS-CoV-2 S300-v3.5 mAb VH
QVQLVQSGAEVKKPGASVKVSCKASGYTFTDYYIHWVRQAPGQGPEWLGYVNQYSGATRYAQKYQGRVTMTRDTSISTAYMQLSRLRPDDTAVYYCARDRPSHEWAMYFFDNWGQGTLVTVSS

SEQ ID NO: 43 - protein, 123 aa, synthetic construct
  REGION 1..123: note = Synthetic sequence SARS-CoV-2 S300-v3.6 mAb VH
QVQLVQSGAEVKKPGASVKVSCKASGYTFTDYYIHWVRQAPGQGPEWLGYVLGYSGATRYAQKYQGRVTMTRDTSISTAYMQLSRLRPDDTAVYYCARDRPSHEWAMYFFDNWGQGTLVTVSS

SEQ ID NO: 44 - protein, 123 aa, synthetic construct
  REGION 1..123: note = Synthetic sequence SARS-CoV-2 S300-v3.7 mAb VH
QVQLVQSGAEVKKPGASVKVSCKASGYTFTDYYIHWVRQAPGQGPEWLGYVTGYSGATRYAQKYQGRVTMTRDTSISTAYMQLSRLRPDDTAVYYCARDRPSHEWAMYFFDNWGQGTLVTVSS

SEQ ID NO: 45 - protein, 123 aa, synthetic construct
  REGION 1..123: note = Synthetic sequence SARS-CoV-2 S300-v3.8 mAb VH
QVQLVQSGAEVKKPGASVKVSCKASGYTFTDYYIHWVRQAPGQGPEWLGYVNGYSGATRYAQKYQGRVTMTRDTSISTAYMQLSRLRPDDTAVYYCARDRPSHEFAMYFFDNWGQGTLVTVSS

SEQ ID NO: 46 - protein, 123 aa, synthetic construct
  REGION 1..123: note = Synthetic sequence SARS-CoV-2 S300-v3.9 mAb VH
QVQLVQSGAEVKKPGASVKVSCKASGYTFTDYYIHWVRQAPGQGPEWLGYVNGYSGATRYAQKYQGRVTMTRDTSISTAYMQLSRLRPDDTAVYYCARDRPSHEYAMYFFDNWGQGTLVTVSS

SEQ ID NO: 47 - protein, 109 aa, synthetic construct
  REGION 1..109: note = Synthetic sequence SARS-CoV-2 S300-v10 mAb VL (VK)
QIVLTQSPGTLSLSPGERATLSCRASQSVPSSYLAWYQQKPGQAPRLLIYGASGRATGIPDRFSGSGSGTDFTLTIRRLEPEDFAVYYCQQYGSSPPLTFGGGTKVEIK

SEQ ID NO: 48 - protein, 109 aa, synthetic construct
  REGION 1..109: note = Synthetic sequence SARS-CoV-2 S300-v11 mAb VL (VK)
QIVLTQSPGTLSLSPGERATLSCRASQSVPSSSLAWYQQKPGQAPRLLIYGASGRATGIPDRFSGSGSGTDFTLTIRRLEPEDFAVYYCQQYGSSPPLTFGGGTKVEIK

SEQ ID NO: 49 - protein, 109 aa, synthetic construct
  REGION 1..109: note = Synthetic sequence SARS-CoV-2 S300-v12 mAb VL (VK)
QIVLTQSPGTLSLSPGERATLSCRASQSVPSSTLAWYQQKPGQAPRLLIYGASGRATGIPDRFSGSGSGTDFTLTIRRLEPEDFAVYYCQQYGSSPPLTFGGGTKVEIK

SEQ ID NO: 50 - protein, 109 aa, synthetic construct
  REGION 1..109: note = Synthetic sequence SARS-CoV-2 S300-v13 mAb VL (VK)
QIVLTQSPGTLSLSPGERATLSCRASQSVPSSALAWYQQKPGQAPRLLIYGASGRATGIPDRFSGSGSGTDFTLTIRRLEPEDFAVYYCQQYGSSPPLTFGGGTKVEIK

SEQ ID NO: 51 - protein, 7 aa, synthetic construct
  REGION 1..7: note = Synthetic sequence SARS-CoV-2 S300-v10 mAb CDRL1
QSVPSSY

SEQ ID NO: 52 - protein, 7 aa, synthetic construct
  REGION 1..7: note = Synthetic sequence SARS-CoV-2 S300-v11 mAb CDRL1
QSVPSSS

SEQ ID NO: 53 - protein, 7 aa, synthetic construct
  REGION 1..7: note = Synthetic sequence SARS-CoV-2 S300-v12 mAb CDRL1
QSVPSST

SEQ ID NO: 54 - protein, 7 aa, synthetic construct
  REGION 1..7: note = Synthetic sequence SARS-CoV-2 S300-v13 mAb CDRL1
QSVPSSA

SEQ ID NO: 55 - protein, 121 aa, synthetic construct
  REGION 1..121: note = Synthetic sequence SARS-CoV-2 S302 mAb VH
QVQLVESGGGVVQPGRSLRLSCAASGFTFSSYGMHWVRQAPGKGLEWVAVISYDGSNKYYADSVKGRFTISRDNSKNTLYLQMNSLRAEDTAVYYCAKDISSGWDRVFDYWGQGTLVTVSS

SEQ ID NO: 56 - protein, 8 aa, synthetic construct
  REGION 1..8: note = Synthetic sequence SARS-CoV-2 S302 mAb CDRH1
GFTFSSYG

SEQ ID NO: 57 - protein, 8 aa, synthetic construct
  REGION 1..8: note = Synthetic sequence SARS-CoV-2 S302 mAb CDRH2
ISYDGSNK

SEQ ID NO: 58 - protein, 14 aa, synthetic construct
  REGION 1..14: note = Synthetic sequence SARS-CoV-2 S302 mAb CDRH3
AKDISSGWDRVFDY

SEQ ID NO: 59 - protein, 108 aa, synthetic construct
  REGION 1..108: note = Synthetic sequence SARS-CoV-2 S302 mAb VL (VK)
EILLTQSPGTLSLSPGERATLSCRTSQSVGSSYLAWYQQKPGQAPRLLIYAASSRAIGIPDRFSGSGSGTDFTLTISRLEPEDFAVYYCQQYGSSPWTFGQGTKVEIK

SEQ ID NO: 60 - protein, 7 aa, synthetic construct
  REGION 1..7: note = Synthetic sequence SARS-CoV-2 S302 mAb CDRL1
QSVGSSY

SEQ ID NO: 61 - skipped

SEQ ID NO: 62 - protein, 9 aa, synthetic construct
  REGION 1..9: note = Synthetic sequence SARS-CoV-2 S302 mAb CDRL3
QQYGSSPWT

SEQ ID NO: 63 - protein, 124 aa, synthetic construct
  REGION 1..124: note = Synthetic sequence SARS-CoV-2 S303-v1 mAb VH
EVQLVESGGGLVKPGGSLRLSCAASGFTFLTYSMNWVRQTPGKRLQWVSAISGSGGATYYADSVKGRFTISRDNSKNTLYLQMNTVTADDTAIYFCARERDDIFPMGLNAFDIWGQGAMVIVSS

SEQ ID NO: 64 - protein, 8 aa, synthetic construct
  REGION 1..8: note = Synthetic sequence SARS-CoV-2 S303-v1 mAb CDRH1
GFTFLTYS

SEQ ID NO: 65 - protein, 8 aa, synthetic construct
  REGION 1..8: note = Synthetic sequence SARS-CoV-2 S303-v1 mAb CDRH2
ISGSGGAT

SEQ ID NO: 66 - protein, 17 aa, synthetic construct
  REGION 1..17: note = Synthetic sequence SARS-CoV-2 S303-v1 mAb CDRH3
ARERDDIFPMGLNAFDI

SEQ ID NO: 67 - protein, 107 aa, synthetic construct
  REGION 1..107: note = Synthetic sequence SARS-CoV-2 S303-v1 mAb VL (VK)
DIQMTQSPSTLSASVGDRVTITCRASQSISNWLAWYQQKPGKAPKLLIYKASSLESGVPSRFSGSGSGTEFTLTISSLQPDDSATYYCQQYDTYSWTFGQGTKVEIK

SEQ ID NO: 68 - protein, 6 aa, synthetic construct
  REGION 1..6: note = Synthetic sequence SARS-CoV-2 S303-v1 mAb CDRL1
QSISNW

SEQ ID NO: 69 - skipped

SEQ ID NO: 70 - protein, 9 aa, synthetic construct
  REGION 1..9: note = Synthetic sequence SARS-CoV-2 S303-v1 mAb CDRL3
QQYDTYSWT

SEQ ID NO: 71 - protein, 107 aa, synthetic construct
  REGION 1..107: note = Synthetic sequence SARS-CoV-2 S303-v2 mAb VL (VK)
DIQMTQSPSTLSASVGDRVTITCRASQSISNFLAWYQQKPGKAPKLLIYKASSLESGVPSRFSGSGSGTEFTLTISSLQPDDSATYYCQQYDTYSWTFGQGTKVEIK

SEQ ID NO: 72 - protein, 107 aa, synthetic construct
  REGION 1..107: note = Synthetic sequence SARS-CoV-2 S303-v3 mAb VL (VK)
DIQMTQSPSTLSASVGDRVTITCRASQSISNYLAWYQQKPGKAPKLLIYKASSLESGVPSRFSGSGSGTEFTLTISSLQPDDSATYYCQQYDTYSWTFGQGTKVEIK

SEQ ID NO: 73 - protein, 6 aa, synthetic construct
  REGION 1..6: note = Synthetic sequence SARS-CoV-2 S303-v2 mAb CDRL1
QSISNF

SEQ ID NO: 74 - protein, 6 aa, synthetic construct
  REGION 1..6: note = Synthetic sequence SARS-CoV-2 S303-v3 mAb CDRL1
QSISNY

SEQ ID NO: 75 - protein, 107 aa, synthetic construct
  REGION 1..107: note = Synthetic sequence SARS-CoV-2 S303-v4 mAb VL (VK)
DIQMTQSPSTLSASVGDRVTITCRASQSISNWLAWYQQKPGKAPKLLIYKASSLESGVPSRFSGSGSGTEFTLTISSLQPDDSATYYCQQYDTYSFTFGQGTKVEIK

SEQ ID NO: 76 - protein, 107 aa, synthetic construct
  REGION 1..107: note = Synthetic sequence SARS-CoV-2 S303-v5 mAb VL (VK)
DIQMTQSPSTLSASVGDRVTITCRASQSISNWLAWYQQKPGKAPKLLIYKASSLESGVPSRFSGSGSGTEFTLTISSLQPDDSATYYCQQYDTYSYTFGQGTKVEIK

SEQ ID NO: 77 - protein, 9 aa, synthetic construct
  REGION 1..9: note = Synthetic sequence SARS-CoV-2 S303-v4 mAb CDRL3
QQYDTYSFT

SEQ ID NO: 78 - protein, 9 aa, synthetic construct
  REGION 1..9: note = Synthetic sequence SARS-CoV-2 S303-v5 mAb CDRL3
QQYDTYSYT

SEQ ID NO: 79 - protein, 120 aa, synthetic construct
  REGION 1..120: note = Synthetic sequence SARS-CoV-2 S304 mAb VH
EVQLVESGGGLVQPGGSLRLSCAASGFTFSSYDMHWVRQTTGKGLEWVSTIGTAGDTYYPDSVKGRFTISREDAKNSLYLQMNSLRAGDTAVYYCARGDSSGYYYYFDYWGQGTLLTVSS

SEQ ID NO: 80 - protein, 8 aa, synthetic construct
  REGION 1..8: note = Synthetic sequence SARS-CoV-2 S304 mAb CDRH1
GFTFSSYD

SEQ ID NO: 81 - protein, 7 aa, synthetic construct
  REGION 1..7: note = Synthetic sequence SARS-CoV-2 S304 mAb CDRH2
IGTAGDT

SEQ ID NO: 82 - protein, 14 aa, synthetic construct
  REGION 1..14: note = Synthetic sequence SARS-CoV-2 S304 mAb CDRH3
ARGDSSGYYYYFDY

SEQ ID NO: 83 - protein, 108 aa, synthetic construct
  REGION 1..108: note = Synthetic sequence SARS-CoV-2 S304 mAb VL (VK)
DIQMTQSPSSLSAAVGDRVTITCRASQSIGSYLNWYQQKPGKAPKLLIYAASSLQSGVPSRFSGSGSGTDFTLTISSLQPEDFAIYYCQQSYVSPTYTFGPGTKVDIK

SEQ ID NO: 84 - protein, 6 aa, synthetic construct
  REGION 1..6: note = Synthetic sequence SARS-CoV-2 S304 mAb CDRL1
QSIGSY

SEQ ID NO: 85 - skipped

SEQ ID NO: 86 - protein, 10 aa, synthetic construct
  REGION 1..10: note = Synthetic sequence SARS-CoV-2 S304 mAb CDRL3
QQSYVSPTYT

SEQ ID NO: 87 - protein, 123 aa, synthetic construct
  REGION 1..123: note = Synthetic sequence SARS-CoV-2 S306 mAb VH
QVQLVQSGAEVKKPGASVKVSCKASTYTFTSFGISWVRQAPGQGLEWMGWITTYSGDTNYAQKFQGRVTMTTDTSTNTAYMELRSLRSDDTAVYYCASDYFDSSGYYHSFDYWGQGTLVTVSS

SEQ ID NO: 88 - protein, 8 aa, synthetic construct
  REGION 1..8: note = Synthetic sequence SARS-CoV-2 S306 mAb CDRH1
TYTFTSFG

SEQ ID NO: 89 - protein, 8 aa, synthetic construct
  REGION 1..8: note = Synthetic sequence SARS-CoV-2 S306 mAb CDRH2
ITTYSGDT

SEQ ID NO: 90 - protein, 16 aa, synthetic construct
  REGION 1..16: note = Synthetic sequence SARS-CoV-2 S306 mAb CDRH3
ASDYFDSSGYYHSFDY

SEQ ID NO: 91 - protein, 109 aa, synthetic construct
  REGION 1..109: note = Synthetic sequence SARS-CoV-2 S306 mAb VL (VK)
EIVLTQSPDTLSLSPGERATLSCRASQSVSSYLAWYQQRPGQAPRLLIYDASKRATGIPARFSGSGSGTDFTLTISSLEPEDFAVYYCQQRSNWPPGCSFGQGTKVEIK

SEQ ID NO: 92 - protein, 6 aa, synthetic construct
  REGION 1..6: note = Synthetic sequence SARS-CoV-2 S306 mAb CDRL1
QSVSSY

SEQ ID NO: 93 - skipped

SEQ ID NO: 94 - protein, 11 aa, synthetic construct
  REGION 1..11: note = Synthetic sequence SARS-CoV-2 S306 mAb CDRL3
QQRSNWPPGCS

SEQ ID NO: 95 - protein, 127 aa, synthetic construct
  REGION 1..127: note = Synthetic sequence SARS-CoV-2 S308-v1 mAb VH
QVQLVESGGGVVQPGRSLRLSCAASRFTFSSYGMHWVRQAPGKGLEWVAVIWHDGNNKHYGDSVKGRVTISRDNSKNTLYLQMTSLRAEDTAVYYCARAVTTFKGSGRARMRGMDVWGQGTTVTVSS

SEQ ID NO: 96 - protein, 8 aa, synthetic construct
  REGION 1..8: note = Synthetic sequence SARS-CoV-2 S308-v1 mAb CDRH1
RFTFSSYG

SEQ ID NO: 97 - protein, 8 aa, synthetic construct
  REGION 1..8: note = Synthetic sequence SARS-CoV-2 S308-v1 mAb CDRH2
IWHDGNNK

SEQ ID NO: 98 - protein, 20 aa, synthetic construct
  REGION 1..20: note = Synthetic sequence SARS-CoV-2 S308-v1 mAb CDRH3
ARAVTTFKGSGRARMRGMDV

SEQ ID NO: 99 - protein, 107 aa, synthetic construct
  REGION 1..107: note = Synthetic sequence SARS-CoV-2 S308-v1 mAb VL (VK)
DIQLTQSPSFLSASVGDRVTITCRASQGINTYLAWYQQKPGKAPKLLIYAASTLQSGVPSRFSGSGSGTEFTLTISSLQPEDFATYYCQHLDTYPFTFGPGTKVDIK

SEQ ID NO: 100 - protein, 6 aa, synthetic construct
  REGION 1..6: note = Synthetic sequence SARS-CoV-2 S308-v1 mAb CDRL1
QGINTY

SEQ ID NO: 101 - skipped

SEQ ID NO: 102 - protein, 9 aa, synthetic construct
  REGION 1..9: note = Synthetic sequence SARS-CoV-2 S308-v1 mAb CDRL3
QHLDTYPFT

SEQ ID NO: 103 - protein, 127 aa, synthetic construct
  REGION 1..127: note = Synthetic sequence SARS-CoV-2 S308-v2 mAb VH
QVQLVESGGGVVQPGRSLRLSCAASRFTFSSYGMHWVRQAPGKGLEWVAVIWHDGNNKHYGDSVKGRVTISRDNSKNTLYLQMTSLRAEDTAVYYCARAVTTFKGSGRARLRGMDVWGQGTTVTVSS

SEQ ID NO: 104 - protein, 20 aa, synthetic construct
  REGION 1..20: note = Synthetic sequence SARS-CoV-2 S308-v2 mAb CDRH3
ARAVTTFKGSGRARLRGMDV

SEQ ID NO: 105 - protein, 127 aa, synthetic construct [sequence omitted]

SEQ ID NO: 106 - protein, 8 aa, synthetic construct
  REGION 1..8: note = Synthetic sequence SARS-CoV-2 S309-v1 mAb CDRH1
GYPFTSYG

SEQ ID NO: 107 - protein, 8 aa, synthetic construct
  REGION 1..8: note = Synthetic sequence SARS-CoV-2 S309-v1 mAb CDRH2
ISTYNGNT

SEQ ID NO: 108 - protein, 20 aa, synthetic construct
  REGION 1..20: note = Synthetic sequence SARS-CoV-2 S309-v1 mAb CDRH3
ARDYTRGAWFGESLIGGFDN

SEQ ID NO: 109 - protein, 107 aa, synthetic construct
  REGION 1..107: note = Synthetic sequence SARS-CoV-2 S309-v1 mAb VL (VK)
DIQMTQSPSSLSTSVGDRVTITCRASQGINNYVAWYQQKPGKVPKLLIYGASTLQSGVPSRFRGSGSGTGFTLTISSLQPEDVASYYCRKYNSAPWTFGQGTRVEIK

SEQ ID NO: 110 - protein, 6 aa, synthetic construct
  REGION 1..6: note = Synthetic sequence SARS-CoV-2 S309-v1 mAb CDRL1
QGINNY

SEQ ID NO: 111 - skipped

SEQ ID NO: 112 - protein, 9 aa, synthetic construct
  REGION 1..9: note = Synthetic sequence SARS-CoV-2 S309-v1 mAb CDRL3
RKYNSAPWT

SEQ ID NO: 113 - protein, 127 aa, synthetic construct
  REGION 1..127: note = Synthetic sequence SARS-CoV-2 S309-v1.1 mAb VH
QVQLVQSGAEVKKPGASVKVSCKASGYPFTSYGISWVRQAPGQGLEWMGWISTYQGNTNYAQKFQGRVTMTTDTSTTTGYMELRRLRSDDTAVYYCARDYTRGAWFGESLIGGFDNWGQGTLVTVSS

SEQ ID NO: 114 - protein, 127 aa, synthetic construct
  REGION 1..127: note = Synthetic sequence SARS-CoV-2 S309-v1.2 mAb VH
QVQLVQSGAEVKKPGASVKVSCKASGYPFTSYGISWVRQAPGQGLEWMGWISTYNSNTNYAQKFQGRVTMTTDTSTTTGYMELRRLRSDDTAVYYCARDYTRGAWFGESLIGGFDNWGQGTLVTVSS

SEQ ID NO: 115 - protein, 127 aa, synthetic construct
  REGION 1..127: note = Synthetic sequence SARS-CoV-2 S309-v1.3 mAb VH
QVQLVQSGAEVKKPGASVKVSCKASGYPFTSYGISWVRQAPGQGLEWMGWISTYNANTNYAQKFQGRVTMTTDTSTTTGYMELRRLRSDDTAVYYCARDYTRGAWFGESLIGGFDNWGQGTLVTVSS

SEQ ID NO: 116 - protein, 127 aa, synthetic construct
  REGION 1..127: note = Synthetic sequence SARS-CoV-2 S309-v1.4 mAb VH
QVQLVQSGAEVKKPGASVKVSCKASGYPFTSYGISWVRQAPGQGLEWMGWISTYNQNTNYAQKFQGRVTMTTDTSTTTGYMELRRLRSDDTAVYYCARDYTRGAWFGESLIGGFDNWGQGTLVTVSS

SEQ ID NO: 117 - protein, 127 aa, synthetic construct
  REGION 1..127: note = Synthetic sequence SARS-CoV-2 S309-v1.5 mAb VH
QVQLVQSGAEVKKPGASVKVSCKASGYPFTSYGISWVRQAPGQGLEWMGWISTYLGNTNYAQKFQGRVTMTTDTSTTTGYMELRRLRSDDTAVYYCARDYTRGAWFGESLIGGFDNWGQGTLVTVSS

SEQ ID NO: 118 - protein, 127 aa, synthetic construct
  REGION 1..127: note = Synthetic sequence SARS-CoV-2 S309-v1.6 mAb VH
QVQLVQSGAEVKKPGASVKVSCKASGYPFTSYGISWVRQAPGQGLEWMGWISTYTGNTNYAQKFQGRVTMTTDTSTTTGYMELRRLRSDDTAVYYCARDYTRGAWFGESLIGGFDNWGQGTLVTVSS

SEQ ID NO: 119 - protein, 127 aa, synthetic construct
  REGION 1..127: note = Synthetic sequence SARS-CoV-2 S309-v1.7 mAb VH
QVQLVQSGAEVKKPGASVKVSCKASGYPFTSYGISWVRQAPGQGLEWMGWISTYNGNTNYAQKFQGRVTMTTDTSTTTGYMELRRLRSDDTAVYYCARDYTRGAFFGESLIGGFDNWGQGTLVTVSS

SEQ ID NO: 120 - protein, 127 aa, synthetic construct
  REGION 1..127: note = Synthetic sequence SARS-CoV-2 S309-v1.8 mAb VH
QVQLVQSGAEVKKPGASVKVSCKASGYPFTSYGISWVRQAPGQGLEWMGWISTYNGNTNYAQKFQGRVTMTTDTSTTTGYMELRRLRSDDTAVYYCARDYTRGAYFGESLIGGFDNWGQGTLVTVSS

SEQ ID NO: 121 - protein, 8 aa, synthetic construct
  REGION 1..8: note = Synthetic sequence SARS-CoV-2 S309-v1.1 mAb CDRH2
ISTYQGNT

SEQ ID NO: 122 - protein, 8 aa, synthetic construct
  REGION 1..8: note = Synthetic sequence SARS-CoV-2 S309-v1.2 mAb CDRH2
ISTYNSNT

SEQ ID NO: 123 - protein, 8 aa, synthetic construct
  REGION 1..8: note = Synthetic sequence SARS-CoV-2 S309-v1.3 mAb CDRH2
ISTYNANT

SEQ ID NO: 124 - protein, 8 aa, synthetic construct
  REGION 1..8: note = Synthetic sequence SARS-CoV-2 S309-v1.4 mAb CDRH2
ISTYNQNT

SEQ ID NO: 125 - protein, 8 aa, synthetic construct
  REGION 1..8: note = Synthetic sequence SARS-CoV-2 S309-v1.5 mAb CDRH2
ISTYLGNT

SEQ ID NO: 126 - protein, 8 aa, synthetic construct
  REGION 1..8: note = Synthetic sequence SARS-CoV-2 S309-v1.6 mAb CDRH2
ISTYTGNT

SEQ ID NO: 127 - protein, 20 aa, synthetic construct
  REGION 1..20: note = Synthetic sequence SARS-CoV-2 S309-v1.7 mAb CDRH3
ARDYTRGAFFGESLIGGFDN

SEQ ID NO: 128 - protein, 20 aa, synthetic construct
  REGION 1..20: note = Synthetic sequence SARS-CoV-2 S309-v1.8 mAb CDRH3
ARDYTRGAYFGESLIGGFDN

SEQ ID NO: 129 - protein, 127 aa, synthetic construct
  REGION 1..127: note = Synthetic sequence SARS-CoV-2 S309-v2 mAb VH
QVQLVQSGAEVKKPGASVKVSCKASGYPFTSYGISWVRQAPGQGLEWMGFISTYNGNTNYAQKFQGRVTMTTDTSTTTGYMELRRLRSDDTAVYYCARDYTRGAWFGESLIGGFDNWGQGTLVTVSS

SEQ ID NO: 130 - protein, 127 aa, synthetic construct
  REGION 1..127: note = Synthetic sequence SARS-CoV-2 S309-v2.1 mAb VH
QVQLVQSGAEVKKPGASVKVSCKASGYPFTSYGISWVRQAPGQGLEWMGFISTYQGNTNYAQKFQGRVTMTTDTSTTTGYMELRRLRSDDTAVYYCARDYTRGAWFGESLIGGFDNWGQGTLVTVSS

SEQ ID NO: 131 - protein, 127 aa, synthetic construct
  REGION 1..127: note = Synthetic sequence SARS-CoV-2 S309-v2.2 mAb VH
QVQLVQSGAEVKKPGASVKVSCKASGYPFTSYGISWVRQAPGQGLEWMGFISTYNSNTNYAQKFQGRVTMTTDTSTTTGYMELRRLRSDDTAVYYCARDYTRGAWFGESLIGGFDNWGQGTLVTVSS

SEQ ID NO: 132 - protein, 127 aa, synthetic construct
  REGION 1..127: note = Synthetic sequence SARS-CoV-2 S309-v2.3 mAb VH
QVQLVQSGAEVKKPGASVKVSCKASGYPFTSYGISWVRQAPGQGLEWMGFISTYNANTNYAQKFQGRVTMTTDTSTTTGYMELRRLRSDDTAVYYCARDYTRGAWFGESLIGGFDNWGQGTLVTVSS

SEQ ID NO: 133 - protein, 127 aa, synthetic construct
  REGION 1..127: note = Synthetic sequence SARS-CoV-2 S309-v2.4 mAb VH
QVQLVQSGAEVKKPGASVKVSCKASGYPFTSYGISWVRQAPGQGLEWMGFISTYNQNTNYAQKFQGRVTMTTDTSTTTGYMELRRLRSDDTAVYYCARDYTRGAWFGESLIGGFDNWGQGTLVTVSS

SEQ ID NO: 134 - protein, 127 aa, synthetic construct
  REGION 1..127: note = Synthetic sequence SARS-CoV-2 S309-v2.5 mAb VH
QVQLVQSGAEVKKPGASVKVSCKASGYPFTSYGISWVRQAPGQGLEWMGFISTYLGNTNYAQKFQGRVTMTTDTSTTTGYMELRRLRSDDTAVYYCARDYTRGAWFGESLIGGFDNWGQGTLVTVSS

SEQ ID NO: 135 - protein, 127 aa, synthetic construct
  REGION 1..127: note = Synthetic sequence SARS-CoV-2 S309-v2.6 mAb VH
QVQLVQSGAEVKKPGASVKVSCKASGYPFTSYGISWVRQAPGQGLEWMGFISTYTGNTNYAQKFQGRVTMTTDTSTTTGYMELRRLRSDDTAVYYCARDYTRGAWFGESLIGGFDNWGQGTLVTVSS

SEQ ID NO: 136 - protein, 127 aa, synthetic construct
  REGION 1..127: note = Synthetic sequence SARS-CoV-2 S309-v2.7 mAb VH
QVQLVQSGAEVKKPGASVKVSCKASGYPFTSYGISWVRQAPGQGLEWMGFISTYNGNTNYAQKFQGRVTMTTDTSTTTGYMELRRLRSDDTAVYYCARDYTRGAFFGESLIGGFDNWGQGTLVTVSS

SEQ ID NO: 137 - protein, 127 aa, synthetic construct
  REGION 1..127: note = Synthetic sequence SARS-CoV-2 S309-v2.8 mAb VH
QVQLVQSGAEVKKPGASVKVSCKASGYPFTSYGISWVRQAPGQGLEWMGFISTYNGNTNYAQKFQGRVTMTTDTSTTTGYMELRRLRSDDTAVYYCARDYTRGAYFGESLIGGFDNWGQGTLVTVSS

SEQ ID NO: 138 - protein, 127 aa, synthetic construct
  REGION 1..127: note = Synthetic sequence SARS-CoV-2 S309-v3 mAb VH
QVQLVQSGAEVKKPGASVKVSCKASGYPFTSYGISWVRQAPGQGLEWMGYISTYNGNTNYAQKFQGRVTMTTDTSTTTGYMELRRLRSDDTAVYYCARDYTRGAWFGESLIGGFDNWGQGTLVTVSS

SEQ ID NO: 139 - protein, 127 aa, synthetic construct
  REGION 1..127: note = Synthetic sequence SARS-CoV-2 S309-v3.1 mAb VH
QVQLVQSGAEVKKPGASVKVSCKASGYPFTSYGISWVRQAPGQGLEWMGYISTYQGNTNYAQKFQGRVTMTTDTSTTTGYMELRRLRSDDTAVYYCARDYTRGAWFGESLIGGFDNWGQGTLVTVSS

SEQ ID NO: 140 - protein, 127 aa, synthetic construct
  REGION 1..127: note = Synthetic sequence SARS-CoV-2 S309-v3.2 mAb VH
QVQLVQSGAEVKKPGASVKVSCKASGYPFTSYGISWVRQAPGQGLEWMGYISTYNSNTNYAQKFQGRVTMTTDTSTTTGYMELRRLRSDDTAVYYCARDYTRGAWFGESLIGGFDNWGQGTLVTVSS

SEQ ID NO: 141 - protein, 127 aa, synthetic construct
  REGION 1..127: note = Synthetic sequence SARS-CoV-2 S309-v3.3 mAb VH
QVQLVQSGAEVKKPGASVKVSCKASGYPFTSYGISWVRQAPGQGLEWMGYISTYNANTNYAQKFQGRVTMTTDTSTTTGYMELRRLRSDDTAVYYCARDYTRGAWFGESLIGGFDNWGQGTLVTVSS

SEQ ID NO: 142 - protein, 127 aa, synthetic construct
  REGION 1..127: note = Synthetic sequence SARS-CoV-2 S309-v3.4 mAb VH
QVQLVQSGAEVKKPGASVKVSCKASGYPFTSYGISWVRQAPGQGLEWMGYISTYNQNTNYAQKFQGRVTMTTDTSTTTGYMELRRLRSDDTAVYYCARDYTRGAWFGESLIGGFDNWGQGTLVTVSS

SEQ ID NO: 143 - protein, 127 aa, synthetic construct
  REGION 1..127: note = Synthetic sequence SARS-CoV-2 S309-v3.5 mAb VH
QVQLVQSGAEVKKPGASVKVSCKASGYPFTSYGISWVRQAPGQGLEWMGYISTYLGNTNYAQKFQGRVTMTTDTSTTTGYMELRRLRSDDTAVYYCARDYTRGAWFGESLIGGFDNWGQGTLVTVSS

SEQ ID NO: 144 - protein, 127 aa, synthetic construct
  REGION 1..127: note = Synthetic sequence SARS-CoV-2 S309-v3.6 mAb VH
QVQLVQSGAEVKKPGASVKVSCKASGYPFTSYGISWVRQAPGQGLEWMGYISTYTGNTNYAQKFQGRVTMTTDTSTTTGYMELRRLRSDDTAVYYCARDYTRGAWFGESLIGGFDNWGQGTLVTVSS

SEQ ID NO: 145 - protein, 127 aa, synthetic construct
  REGION 1..127: note = Synthetic sequence SARS-CoV-2 S309-v3.7 mAb VH
QVQLVQSGAEVKKPGASVKVSCKASGYPFTSYGISWVRQAPGQGLEWMGYISTYNGNTNYAQKFQGRVTMTTDTSTTTGYMELRRLRSDDTAVYYCARDYTRGAFFGESLIGGFDNWGQGTLVTVSS

SEQ ID NO: 146 - protein, 127 aa, synthetic construct
  REGION 1..127: note = Synthetic sequence SARS-CoV-2 S309-v3.8 mAb VH
QVQLVQSGAEVKKPGASVKVSCKASGYPFTSYGISWVRQAPGQGLEWMGYISTYNGNTNYAQKFQGRVTMTTDTSTTTGYMELRRLRSDDTAVYYCARDYTRGAYFGESLIGGFDNWGQGTLVTVSS

SEQ ID NO: 147 - protein, 107 aa, synthetic construct
  REGION 1..107: note = Synthetic sequence SARS-CoV-2 S309-v9 mAb VL (VK)
DIQMTQSPSSLSTSVGDRVTITCRASQGINNYVAWYQQKPGKVPKLLIYGASTLQSGVPSRFRGSGSGTGFTLTISSLQPEDVASYYCRKYNSAPGTFGQGTRVEIK

SEQ ID NO: 148 - protein, 107 aa, synthetic construct
  REGION 1..107: note = Synthetic sequence SARS-CoV-2 S309-v10 mAb VL (VK)
DIQMTQSPSSLSTSVGDRVTITCRASQGINNYVAWYQQKPGKVPKLLIYGASTLQSGVPSRFRGSGSGTGFTLTISSLQPEDVASYYCRKYNSAPRTFGQGTRVEIK

SEQ ID NO: 149 - protein, 107 aa, synthetic construct
  REGION 1..107: note = Synthetic sequence SARS-CoV-2 S309-v11 mAb VL (VK)
DIQMTQSPSSLSTSVGDRVTITCRASQGINNYVAWYQQKPGKVPKLLIYGASTLQSGVPSRFRGSGSGTGFTLTISSLQPEDVASYYCRKYNSAPFTFGQGTRVEIK

SEQ ID NO: 150 - protein, 107 aa, synthetic construct
  REGION 1..107: note = Synthetic sequence SARS-CoV-2 S309-v12 mAb VL (VK)
DIQMTQSPSSLSTSVGDRVTITCRASQGINNYVAWYQQKPGKVPKLLIYGASTLQSGVPSRFRGSGSGTGFTLTISSLQPEDVASYYCRKYNSAPYTFGQGTRVEIK

SEQ ID NO: 151 - protein, 9 aa, synthetic construct
  REGION 1..9: note = Synthetic sequence SARS-CoV-2 S309-v9 mAb CDRL3
RKYNSAPGT

SEQ ID NO: 152 - protein, 9 aa, synthetic construct
  REGION 1..9: note = Synthetic sequence SARS-CoV-2 S309-v10 mAb CDRL3
RKYNSAPRT

SEQ ID NO: 153 - protein, 9 aa, synthetic construct
  REGION 1..9: note = Synthetic sequence SARS-CoV-2 S309-v11 mAb CDRL3
RKYNSAPFT

SEQ ID NO: 154 - protein, 9 aa, synthetic construct
  REGION 1..9: note = Synthetic sequence SARS-CoV-2 S309-v12 mAb CDRL3
RKYNSAPYT

SEQ ID NO: 155 - protein, 126 aa, synthetic construct
  REGION 1..126: note = Synthetic sequence SARS-CoV-2 S310 mAb VH
QVQLVQSGAELKKPGSSVKVSCKASGGTFNSYSFNWVRQAPGQGLEWLGGIIPVLGTSNYAQKFQGRVAVTADEFTTTAYMELSSLRSEDTAVYYCATRTYDSSGYRPYYYGLDVWGQGTPVTVSS

SEQ ID NO: 156 - protein, 8 aa, synthetic construct
  REGION 1..8: note = Synthetic sequence SARS-CoV-2 S310 mAb CDRH1
GGTFNSYS

SEQ ID NO: 157 - protein, 8 aa, synthetic construct
  REGION 1..8: note = Synthetic sequence SARS-CoV-2 S310 mAb CDRH2
IIPVLGTS

SEQ ID NO: 158 - protein, 19 aa, synthetic construct
  REGION 1..19: note = Synthetic sequence SARS-CoV-2 S310 mAb CDRH3
ATRTYDSSGYRPYYYGLDV

SEQ ID NO: 159 - protein, 110 aa, synthetic construct
  REGION 1..110: note = Synthetic sequence SARS-CoV-2 S310 mAb VL (VK)
QSALTQPASVSGSPGQSITISCTGTSSDVGSYNLVSWYQQRPGKAPELMIYEVTKRPSGLSNRFSGSKSGNTASLTISGLQAEDEADYYCCSYAGSDTVIFGGGTKVTVL

SEQ ID NO: 160 - protein, 9 aa, synthetic construct
  REGION 1..9: note = Synthetic sequence SARS-CoV-2 S310 mAb CDRL1
SSDVGSYNL

SEQ ID NO: 161 - skipped

SEQ ID NO: 162 - protein, 10 aa, synthetic construct
  REGION 1..10: note = Synthetic sequence SARS-CoV-2 S310 mAb CDRL3
CSYAGSDTVI

SEQ ID NO: 163 - DNA, 29902 bp, betacoronavirus SARS coronavirus 2
  source 1..29902: mol_type = genomic DNA
attaaaggtttataccttcccaggtaacaaaccaaccaactttcgatctcttgtagatctgttctctaaacgaactttaaaatctgtgtggctgtcactcggctgcatgcttagtgcactcacgcagtataattaataactaattactgtcgttgacaggacacgagtaactcgtctatcttctgcaggctgcttacggtttcgtccgtgttgcagccgatcatcagcacatctaggtttcgtccgggtgtgaccgaaaggtaagatggagagccttgtccctggtttcaacgagaaaacacacgtccaactcagtttgcctgttttacaggttcgcgacgtgctcgtacgtggctttggagactccgtggaggaggtcttatcagaggccgtcaacatcttaaagatggcacttgtggcttagtagaagttgaaaaaggcgttttgcctcaacttgaacagccctatgtgttcatcaaacgttcggatgctcgaactgcacctcatggtcatgttatggttgagctggtagcagaactcgaaggcattcagtacggtcgtagtggtgagacacttggtgtccttgtccctcatgtgggcgaaataccagtggcttaccgcaaggttcttcttcgtaagaacggtaataaaggagctggtggccatagttacggcgccgatctaaagtcatttgacttaggcgacgagcttggcactgatccttatgaagattttcaagaaaactggaacactaaacatagcagtggtgttacccgtgaactcatgcgtgagcttaacggaggggcatacactcgctatgtcgataacaacttctgtggccctgatggctaccctcttgagtgcattaaagaccttctagcacgtgctggtaaagcttcatgcactttgtccgaacaactggactttattgacactaagaggggtgtatactgctgccgtgaacatgagcatgaaattgcttggtacacggaacgttctgaaaagagctatgaattgcagacaccttttgaaattaaattggcaaagaaatttgacaccttcaatggggaatgtccaaattttgtatttcccttaaattccataatcaagactattcaaccaagggttgaaaagaaaaagcttgatggctttatgggtagaattcgatctgtctatccagttgcgtcaccaaatgaatgcaaccaaatgtgcctttcaactctcatgaagtgtgatcattgtggtgaaacttcatggcagacgggcgattttgttaaagccacttgcgaattttgtggcactgagaatttgactaaagaaggtgccactacttgtggttacttaccccaaaatgctgttgttaaaatttattgtccagcatgtcacaattcagaagtaggacctgagcatagtcttgccgaataccataatgaatctggcttgaaaaccattcttcgtaagggtggtcgcactattgcctttggaggctgtgtgttctcttatgttggttgccataacaagtgtgcctattgggttccacgtgctagcgctaacataggttgtaaccatacaggtgttgttggagaaggttccgaaggtcttaatgacaaccttcttgaaatactccaaaaagagaaagtcaacatcaatattgttggtgactttaaacttaatgaagagatcgccattattttggcatctttttctgcttccacaagtgcttttgtggaaactgtgaaaggtttggattataaagcattcaaacaaattgttgaatcctgtggtaattttaaagttacaaaaggaaaagctaaaaaaggtgcctggaatattggtgaacagaaatcaatactgagtcctctttatgcatttgcatcagaggctgctcgtgttgtacgatcaattttctcccgcactcttgaaactgctcaaaattctgtgcgtgttttacagaaggccgctataacaatactagatggaatttcacagtattcactgagactcattgatgctatgatgttcacatctgatttggctactaacaatctagttgtaatggcctacattacaggtggtgttgttcagttgacttcgcagtggctaactaacatctttggcactgtttatgaaaaactcaaacccgtccttgattggcttgaagagaagtttaaggaaggtgtagagtttcttagagacggttgggaaattgttaaatttatctcaacctgtgcttgtgaaattgtcggtggacaaattgtcacctgtgcaaaggaaattaaggagagtgttcagacattctttaagcttgtaaataaatttttggctttgtgtgctgactctatcattattggtggagctaaacttaaagccttgaatttaggtgaaacatttgtcacgcactcaaagggattgtacagaaagtgtgttaaatccagagaagaaactggcctactcatgcctctaaaagccccaaaagaaattatcttcttagagggagaaacacttcccacagaagtgttaacagaggaagttgtcttgaaaactggtgatttacaaccattagaacaacctactagtgaagctgttgaagctccattggttggtacaccagtttgtattaacgggcttatgttgctcgaaatcaaagacacagaaaagtactgtgcccttgcacctaatatgatggtaacaaacaataccttcacactcaaaggcggtgcaccaacaaaggttacttttggtgatgacactgtgatagaagtgcaaggttacaagagtgtgaatatcacttttgaacttgatgaaaggattgataaagtacttaatgagaagtgctctgcctatacagttgaactcggtacagaagtaaatgagttcgcctgtgttgtggcagatgctgtcataaaaactttgcaaccagtatctgaattacttacaccactgggcattgatttagatgagtggagtatggctacatactacttatttgatgagtctggtgagtttaaattggcttcacatatgtattgttctttctaccctccagatgaggatgaagaagaaggtgattgtgaagaagaagagtttgagccatcaactcaatatgagtatggtactgaagatgattaccaaggtaaacctttggaatttggtgccacttctgctgctcttcaacctgaagaagagcaagaagaagattggttagatgatgatagtcaacaaactgttggtcaacaagacggcagtgaggacaatcagacaactactattcaaacaattgttgaggttcaacctcaattagagatggaacttacaccagttgttcagactattgaagtgaatagttttagtggttatttaaaacttactgacaatgtatacattaaaaatgcagacattgtggaagaagctaaaaaggtaaaaccaacagtggttgttaatgcagccaatgtttaccttaaacatggaggaggtgttgcaggagccttaaataaggctactaacaatgccatgcaagttgaatctgatgattacatagctactaatggaccacttaaagtgggtggtagttgtgttttaagcggacacaatcttgctaaacactgtcttcatgttgtcggcccaaatgttaacaaaggtgaagacattcaacttcttaagagtgcttatgaaaattttaatcagcacgaagttctacttgcaccattattatcagctggtatttttggtgctgaccctatacattctttaagagtttgtgtagatactgttcgcacaaatgtctacttagctgtctttgataaaaatctctatgacaaacttgtttcaagctttttggaaatgaagagtgaaaagcaagttgaacaaaagatcgctgagattcctaaagaggaagttaagccatttataactgaaagtaaaccttcagttgaacagagaaaacaagatgataagaaaatcaaagcttgtgttgaagaagttacaacaactctggaagaaactaagttcctcacagaaaacttgttactttatattgacattaatggcaatcttcatccagattctgccactcttgttagtgacattgacatcactttcttaaagaaagatgctccatatatagtgggtgatgttgttcaagagggtgttttaactgctgtggttatacctactaaaaaggctggtggcactactgaaatgctagcgaaagctttgagaaaagtgccaacagacaattatataaccacttacccgggtcagggtttaaatggttacactgtagaggaggcaaagacagtgcttaaaaagtgtaaaagtgccttttacattctaccatctattatctctaatgagaagcaagaaattcttggaactgtttcttggaatttgcgagaaatgcttgcacatgcagaagaaacacgcaaattaatgcctgtctgtgtggaaactaaagccatagtttcaactatacagcgtaaatataagggtattaaaatacaagagggtgtggttgattatggtgctagattttacttttacaccagtaaaacaactgtagcgtcacttatcaacacacttaacgatctaaatgaaactcttgttacaatgccacttggctatgtaacacatggcttaaatttggaagaagctgctcggtatatgagatctctcaaagtgccagctacagtttctgtttcttcacctgatgctgttacagcgtataatggttatcttacttcttcttctaaaacacctgaagaacattttattgaaaccatctcacttgctggttcctataaagattggtcctattctggacaatctacacaactaggtatagaatttcttaagagaggtgataaaagtgtatattacactagtaatcctaccacattccacctagatggtgaagttatcacctttgacaatcttaagacacttctttctttgagagaagtgaggactattaaggtgtttacaacagtagacaacattaacctccacacgcaagttgtggacatgtcaatgacatatggacaacagtttggtccaacttatttggatggagctgatgttactaaaataaaacctcataattcacatgaaggtaaaacattttatgttttacctaatgatgacactctacgtgttgaggcttttgagtactaccacacaactgatcctagttttctgggtaggtacatgtcagcattaaatcacactaaaaagtggaaatacccacaagttaatggtttaacttctattaaatgggcagataacaactgttatcttgccactgcattgttaacactccaacaaatagagttgaagtttaatccacctgctctacaagatgcttattacagagcaagggctggtgaagctgctaacttttgtgcacttatcttagcctactgtaataagacagtaggtgagttaggtgatgttagagaaacaatgagttacttgtttcaacatgccaatttagattcttgcaaaagagtcttgaacgtggtgtgtaaaacttgtggacaacagcagacaacccttaagggtgtagaagctgttatgtacatgggcacactttcttatgaacaatttaagaaaggtgttcagataccttgtacgtgtggtaaacaagctacaaaatatctagtacaacaggagtcaccttttgttatgatgtcagcaccacctgctcagtatgaacttaagcatggtacatttacttgtgctagtgagtacactggtaattaccagtgtggtcactataaacatataacttctaaagaaactttgtattgcatagacggtgctttacttacaaagtcctcagaatacaaaggtcctattacggatgttttctacaaagaaaacagttacacaacaaccataaaaccagttacttataaattggatggtgttgtttgtacagaaattgaccctaagttggacaattattataagaaagacaattcttatttcacagagcaaccaattgatcttgtaccaaaccaaccatatccaaacgcaagcttcgataattttaagtttgtatgtgataatatcaaatttgctgatgatttaaaccagttaactggttataagaaacctgcttcaagagagcttaaagttacatttttccctgacttaaatggtgatgtggtggctattgattataaacactacacaccctcttttaagaaaggagctaaattgttacataaacctattgtttggcatgttaacaatgcaactaataaagccacgtataaaccaaatacctggtgtatacgttgtctttggagcacaaaaccagttgaaacatcaaattcgtttgatgtactgaagtcagaggacgcgcagggaatggataatcttgcctgcgaagatctaaaaccagtctctgaagaagtagtggaaaatcctaccatacagaaagacgttcttgagtgtaatgtgaaaactaccgaagttgtaggagacattatacttaaaccagcaaataatagtttaaaaattacagaagaggttggccacacagatctaatggctgcttatgtagacaattctagtcttactattaagaaacctaatgaattatctagagtattaggtttgaaaacccttgctactcatggtttagctgctgttaatagtgtcccttgggatactatagctaattatgctaagccttttcttaacaaagttgttagtacaactactaacatagttacacggtgtttaaaccgtgtttgtactaattatatgccttatttctttactttattgctacaattgtgtacttttactagaagtacaaattctagaattaaagcatctatgccgactactatagcaaagaatactgttaagagtgtcggtaaattttgtctagaggcttcatttaattatttgaagtcacctaatttttctaaactgataaatattataatttggtttttactattaagtgtttgcctaggttctttaatctactcaaccgctgctttaggtgttttaatgtctaatttaggcatgccttcttactgtactggttacagagaaggctatttgaactctactaatgtcactattgcaacctactgtactggttctataccttgtagtgtttgtcttagtggtttagattctttagacacctatccttctttagaaactatacaaattaccatttcatcttttaaatgggatttaactgcttttggcttagttgcagagtggtttttggcatatattcttttcactaggtttttctatgtacttggattggctgcaatcatgcaattgtttttcagctattttgcagtacattttattagtaattcttggcttatgtggttaataattaatcttgtacaaatggccccgatttcagctatggttagaatgtacatcttctttgcatcattttattatgtatggaaaagttatgtgcatgttgtagacggttgtaattcatcaacttgtatgatgtgttacaaacgtaatagagcaacaagagtcgaatgtacaactattgttaatggtgttagaaggtccttttatgtctatgctaatggaggtaaaggcttttgcaaactacacaattggaattgtgttaattgtgatacattctgtgctggtagtacatttattagtgatgaagttgcgagagacttgtcactacagtttaaaagaccaataaatcctactgaccagtcttcttacatcgttgatagtgttacagtgaagaatggttccatccatctttactttgataaagctggtcaaaagacttatgaaagacattctctctctcattttgttaacttagacaacctgagagctaataacactaaaggttcattgcctattaatgttatagtttttgatggtaaatcaaaatgtgaagaatcatctgcaaaatcagcgtctgtttactacagtcagcttatgtgtcaacctatactgttactagatcaggcattagtgtctgatgttggtgatagtgcggaagttgcagttaaaatgtttgatgcttacgttaatacgttttcatcaacttttaacgtaccaatggaaaaactcaaaacactagttgcaactgcagaagctgaacttgcaaagaatgtgtccttagacaatgtcttatctacttttatttcagcagctcggcaagggtttgttgattcagatgtagaaactaaagatgttgttgaatgtcttaaattgtcacatcaatctgacatagaagttactggcgatagttgtaataactatatgctcacctataacaaagttgaaaacatgacaccccgtgaccttggtgcttgtattgactgtagtgcgcgtcatattaatgcgcaggtagcaaaaagtcacaacattgctttgatatggaacgttaaagatttcatgtcattgtctgaacaactacgaaaacaaatacgtagtgctgctaaaaagaataacttaccttttaagttgacatgtgcaactactagacaagttgttaatgttgtaacaacaaagatagcacttaagggtggtaaaattgttaataattggttgaagcagttaattaaagttacacttgtgttcctttttgttgctgctattttctatttaataacacctgttcatgtcatgtctaaacatactgacttttcaagtgaaatcataggatacaaggctattgatggtggtgtcactcgtgacatagcatctacagatacttgttttgctaacaaacatgctgattttgacacatggtttagccagcgtggtggtagttatactaatgacaaagcttgcccattgattgctgcagtcataacaagagaagtgggttttgtcgtgcctggtttgcctggcacgatattacgcacaactaatggtgactttttgcatttcttacctagagtttttagtgcagttggtaacatctgttacacaccatcaaaacttatagagtacactgactttgcaacatcagcttgtgttttggctgctgaatgtacaatttttaaagatgcttctggtaagccagtaccatattgttatgataccaatgtactagaaggttctgttgcttatgaaagtttacgccctgacacacgttatgtgctcatggatggctctattattcaatttcctaacacctaccttgaaggttctgttagagtggtaacaacttttgattctgagtactgtaggcacggcacttgtgaaagatcagaagctggtgtttgtgtatctactagtggtagatgggtacttaacaatgattattacagatctttaccaggagttttctgtggtgtagatgctgtaaatttacttactaatatgtttacaccactaattcaacctattggtgctttggacatatcagcatctatagtagctggtggtattgtagctatcgtagtaacatgccttgcctactattttatgaggtttagaagagcttttggtgaatacagtcatgtagttgcctttaatactttactattccttatgtcattcactgtactctgtttaacaccagtttactcattcttacctggtgtttattctgttatttacttgtacttgacattttatcttactaatgatgtttcttttttagcacatattcagtggatggttatgttcacacctttagtacctttctggataacaattgcttatatcatttgtatttccacaaagcatttctattggttctttagtaattacctaaagagacgtgtagtctttaatggtgtttcctttagtacttttgaagaagctgcgctgtgcacctttttgttaaataaagaaatgtatctaaagttgcgtagtgatgtgctattacctcttacgcaatataatagatacttagctctttataataagtacaagtattttagtggagcaatggatacaactagctacagagaagctgcttgttgtcatctcgcaaaggctctcaatgacttcagtaactcaggttctgatgttctttaccaaccaccacaaacctctatcacctcagctgttttgcagagtggttttagaaaaatggcattcccatctggtaaagttgagggttgtatggtacaagtaacttgtggtacaactacacttaacggtctttggcttgatgacgtagtttactgtccaagacatgtgatctgcacctctgaagacatgcttaaccctaattatgaagatttactcattcgtaagtctaatcataatttcttggtacaggctggtaatgttcaactcagggttattggacattctatgcaaaattgtgtacttaagcttaaggttgatacagccaatcctaagacacctaagtataagtttgttcgcattcaaccaggacagactttttcagtgttagcttgttacaatggttcaccatctggtgtttaccaatgtgctatgaggcccaatttcactattaagggttcattccttaatggttcatgtggtagtgttggttttaacatagattatgactgtgtctctttttgttacatgcaccatatggaattaccaactggagttcatgctggcacagacttagaaggtaacttttatggaccttttgttgacaggcaaacagcacaagcagctggtacggacacaactattacagttaatgttttagcttggttgtacgctgctgttataaatggagacaggtggtttctcaatcgatttaccacaactcttaatgactttaaccttgtggctatgaagtacaattatgaacctctaacacaagaccatgttgacatactaggacctctttctgctcaaactggaattgccgttttagatatgtgtgcttcattaaaagaattactgcaaaatggtatgaatggacgtaccatattgggtagtgctttattagaagatgaatttacaccttttgatgttgttagacaatgctcaggtgttactttccaaagtgcagtgaaaagaacaatcaagggtacacaccactggttgttactcacaattttgacttcacttttagttttagtccagagtactcaatggtctttgttcttttttttgtatgaaaatgcctttttaccttttgctatgggtattattgctatgtctgcttttgcaatgatgtttgtcaaacataagcatgcatttctctgtttgtttttgttaccttctcttgccactgtagcttattttaatatggtctatatgcctgctagttgggtgatgcgtattatgacatggttggatatggttgatactagtttgtctggttttaagctaaaagactgtgttatgtatgcatcagctgtagtgttactaatccttatgacagcaagaactgtgtatgatgatggtgctaggagagtgtggacacttatgaatgtcttgacactcgtttataaagtttattatggtaatgctttagatcaagccatttccatgtgggctcttataatctctgttacttctaactactcaggtgtagttacaactgtcatgtttttggccagaggtattgtttttatgtgtgttgagtattgccctattttcttcataactggtaatacacttcagtgtataatgctagtttattgtttcttaggctatttttgtacttgttactttggcctcttttgtttactcaaccgctactttagactgactcttggtgtttatgattacttagtttctacacaggagtttagatatatgaattcacagggactactcccacccaagaatagcatagatgccttcaaactcaacattaaattgttgggtgttggtggcaaaccttgtatcaaagtagccactgtacagtctaaaatgtcagatgtaaagtgcacatcagtagtcttactctcagttttgcaacaactcagagtagaatcatcatctaaattgtgggctcaatgtgtccagttacacaatgacattctcttagctaaagatactactgaagcctttgaaaaaatggtttcactactttctgttttgctttccatgcagggtgctgtagacataaacaagctttgtgaagaaatgctggacaacagggcaaccttacaagctatagcctcagagtttagttcccttccatcatatgcagcttttgctactgctcaagaagcttatgagcaggctgttgctaatggtgattctgaagttgttcttaaaaagttgaagaagtctttgaatgtggctaaatctgaatttgaccgtgatgcagccatgcaacgtaagttggaaaagatggctgatcaagctatgacccaaatgtataaacaggctagatctgaggacaagagggcaaaagttactagtgctatgcagacaatgcttttcactatgcttagaaagttggataatgatgcactcaacaacattatcaacaatgcaagagatggttgtgttcccttgaacataatacctcttacaacagcagccaaactaatggttgtcataccagactataacacatataaaaatacgtgtgatggtacaacatttacttatgcatcagcattgtgggaaatccaacaggttgtagatgcagatagtaaaattgttcaacttagtgaaattagtatggacaattcacctaatttagcatggcctcttattgtaacagctttaagggccaattctgctgtcaaattacagaataatgagcttagtcctgttgcactacgacagatgtcttgtgctgccggtactacacaaactgcttgcactgatgacaatgcgttagcttactacaacacaacaaagggaggtaggtttgtacttgcactgttatccgatttacaggatttgaaatgggctagattccctaagagtgatggaactggtactatctatacagaactggaaccaccttgtaggtttgttacagacacacctaaaggtcctaaagtgaagtatttatactttattaaaggattaaacaacctaaatagaggtatggtacttggtagtttagctgccacagtacgtctacaagctggtaatgcaacagaagtgcctgccaattcaactgtattatctttctgtgcttttgctgtagatgctgctaaagcttacaaagattatctagctagtgggggacaaccaatcactaattgtgttaagatgttgtgtacacacactggtactggtcaggcaataacagttacaccggaagccaatatggatcaagaatcctttggtggtgcatcgtgttgtctgtactgccgttgccacatagatcatccaaatcctaaaggattttgtgacttaaaaggtaagtatgtacaaatacctacaacttgtgctaatgaccctgtgggttttacacttaaaaacacagtctgtaccgtctgcggtatgtggaaaggttatggctgtagttgtgatcaactccgcgaacccatgcttcagtcagctgatgcacaatcgtttttaaacgggtttgcggtgtaagtgcagcccgtcttacaccgtgcggcacaggcactagtactgatgtcgtatacagggcttttgacatctacaatgataaagtagctggttttgctaaattcctaaaaactaattgttgtcgcttccaagaaaaggacgaagatgacaatttaattgattcttactttgtagttaagagacacactttctctaactaccaacatgaagaaacaatttataatttacttaaggattgtccagctgttgctaaacatgacttctttaagtttagaatagacggtgacatggtaccacatatatcacgtcaacgtcttactaaatacacaatggcagacctcgtctatgctttaaggcattttgatgaaggtaattgtgacacattaaaagaaatacttgtcacatacaattgttgtgatgatgattatttcaataaaaaggactggtatgattttgtagaaaacccagatatattacgcgtatacgccaacttaggtgaacgtgtacgccaagctttgttaaaaacagtacaattctgtgatgccatgcgaaatgctggtattgttggtgtactgacattagataatcaagatctcaatggtaactggtatgatttcggtgatttcatacaaaccacgccaggtagtggagttcctgttgtagattcttattattcattgttaatgcctatattaaccttgaccagggctttaactgcagagtcacatgttgacactgacttaacaaagccttacattaagtgggatttgttaaaatatgacttcacggaagagaggttaaaactctttgaccgttattttaaatattgggatcagacataccacccaaattgtgttaactgtttggatgacagatgcattctgcattgtgcaaactttaatgttttattctctacagtgttcccacctacaagttttggaccactagtgagaaaaatatttgttgatggtgttccatttgtagtttcaactggataccacttcagagagctaggtgttgtacataatcaggatgtaaacttacatagctctagacttagttttaaggaattacttgtgtatgctgctgaccctgctatgcacgctgcttctggtaatctattactagataaacgcactacgtgcttttcagtagctgcacttactaacaatgttgcttttcaaactgtcaaacccggtaattttaacaaagacttctatgactttgctgtgtctaagggtttctttaaggaaggaagttctgttgaattaaaacacttcttctttgctcaggatggtaatgctgctatcagcgattatgactactatcgttataatctaccaacaatgtgtgatatcagacaactactatttgtagttgaagttgttgataagtactttgattgttacgatggtggctgtattaatgctaaccaagtcatcgtcaacaacctagacaaatcagctggttttccatttaataaatggggtaaggctagactttattatgattcaatgagttatgaggatcaagatgcacttttcgcatatacaaaacgtaatgtcatccctactataactcaaatgaatcttaagtatgccattagtgcaaagaatagagctcgcaccgtagctggtgtctctatctgtagtactatgaccaatagacagtttcatcaaaaattattgaaatcaatagccgccactagaggagctactgtagtaattggaacaagcaaattctatggtggttggcacaacatgttaaaaactgtttatagtgatgtagaaaaccctcaccttatgggttgggattatcctaaatgtgatagagccatgcctaacatgcttagaattatggcctcacttgttcttgctcgcaaacatacaacgtgttgtagcttgtcacaccgtttctatagattagctaatgagtgtgctcaagtattgagtgaaatggtcatgtgtggcggttcactatatgttaaaccaggtggaacctcatcaggagatgccacaactgcttatgctaatagtgtttttaacatttgtcaagctgtcacggccaatgttaatgcacttttatctactgatggtaacaaaattgccgataagtatgtccgcaatttacaacacagactttatgagtgtctctatagaaatagagatgttgacacagactttgtgaatgagttttacgcatatttgcgtaaacatttctcaatgatgatactctctgacgatgctgttgtgtgtttcaatagcacttatgcatctcaaggtctagtggctagcataaagaactttaagtcagttctttattatcaaaacaatgtttttatgtctgaagcaaaatgttggactgagactgaccttactaaaggacctcatgaattttgctctcaacatacaatgctagttaaacagggtgatgattatgtgtaccttccttacccagatccatcaagaatcctaggggccggctgttttgtagatgatatcgtaaaaacagatggtacacttatgattgaacggttcgtgtctttagctatagatgcttacccacttactaaacatcctaatcaggagtatgctgatgtctttcatttgtacttacaatacataagaaagctacatgatgagttaacaggacacatgttagacatgtattctgttatgcttactaatgataacacttcaaggtattgggaacctgagttttatgaggctatgtacacaccgcatacagtcttacaggctgttggggcttgtgttctttgcaattcacagacttcattaagatgtggtgcttgcatacgtagaccattcttatgttgtaaatgctgttacgaccatgtcatatcaacatcacataaattagtcttgtctgttaatccgtatgtttgcaatgctccaggttgtgatgtcacagatgtgactcaactttacttaggaggtatgagctattattgtaaatcacataaaccacccattagttttccattgtgtgctaatggacaagtttttggtttatataaaaatacatgtgttggtagcgataatgttactgactttaatgcaattgcaacatgtgactggacaaatgctggtgattacattttagctaacacctgtactgaaagactcaagctttttgcagcagaaacgctcaaagctactgaggagacatttaaactgtcttatggtattgctactgtacgtgaagtgctgtctgacagagaattacatctttcatgggaagttggtaaacctagaccaccacttaaccgaaattatgtctttactggttatcgtgtaactaaaaacagtaaagtacaaataggagagtacacctttgaaaaaggtgactatggtgatgctgttgtttaccgaggtacaacaacttacaaattaaatgttggtgattattttgtgctgacatcacatacagtaatgccattaagtgcacctacactagtgccacaagagcactatgttagaattactggcttatacccaacactcaatatctcagatgagttttctagcaatgttgcaaattatcaaaaggttggtatgcaaaagtattctacactccagggaccacctggtactggtaagagtcattttgctattggcctagctctctactacccttctgctcgcatagtgtatacagcttgctctcatgccgctgttgatgcactatgtgagaaggcattaaaatatttgcctatagataaatgtagtagaattatacctgcacgtgctcgtgtagagtgttttgataaattcaaagtgaattcaacattagaacagtatgtcttttgtactgtaaatgcattgcctgagacgacagcagatatagttgtctttgatgaaatttcaatggccacaaattatgatttgagtgttgtcaatgccagattacgtgctaagcactatgtgtacattggcgaccctgctcaattacctgcaccacgcacattgctaactaagggcacactagaaccagaatatttcaattcagtgtgtagacttatgaaaactataggtccagacatgttcctcggaacttgtcggcgttgtcctgctgaaattgttgacactgtgagtgctttggtttatgataataagcttaaagcacataaagacaaatcagctcaatgctttaaaatgttttataagggtgttatcacgcatgatgtttcatctgcaattaacaggccacaaataggcgtggtaagagaattccttacacgtaaccctgcttggagaaaagctgtctttatttcaccttataattcacagaatgctgtagcctcaaagattttgggactaccaactcaaactgttgattcatcacagggctcagaatatgactatgtcatattcactcaaaccactgaaacagctcactcttgtaatgtaaacagatttaatgttgctattaccagagcaaaagtaggcatactttgcataatgtctgatagagacctttatgacaagttgcaatttacaagtcttgaaattccacgtaggaatgtggcaactttacaagctgaaaatgtaacaggactctttaaagattgtagtaaggtaatcactgggttacatcctacacaggcacctacacacctcagtgttgacactaaattcaaaactgaaggtttatgtgttgacatacctggcatacctaaggacatgacctatagaagactcatctctatgatgggttttaaaatgaattatcaagttaatggttaccctaacatgtttatcacccgcgaagaagctataagacatgtacgtgcatggattggcttcgatgtcgaggggtgtcatgctactagagaagctgttggtaccaatttacctttacagctaggtttttctacaggtgttaacctagttgctgtacctacaggttatgttgatacacctaataatacagatttttccagagttagtgctaaaccaccgcctggagatcaatttaaacacctcataccacttatgtacaaaggacttccttggaatgtagtgcgtataaagattgtacaaatgttaagtgacacacttaaaaatctctctgacagagtcgtatttgtcttatgggcacatggctttgagttgacatctatgaagtattttgtgaaaataggacctgagcgcacctgttgtctatgtgatagacgtgccacatgcttttccactgcttcagacacttatgcctgttggcatcattctattggatttgattacgtctataatccgtttatgattgatgttcaacaatggggttttacaggtaacctacaaagcaaccatgatctgtattgtcaagtccatggtaatgcacatgtagctagttgtgatgcaatcatgactaggtgtctagctgtccacgagtgctttgttaagcgtgttgactggactattgaatatcctataattggtgatgaactgaagattaatgcggcttgtagaaaggttcaacacatggttgttaaagctgcattattagcagacaaattcccagttcttcacgacattggtaaccctaaagctattaagtgtgtacctcaagctgatgtagaatggaagttctatgatgcacagccttgtagtgacaaagcttataaaatagaagaattattctattcttatgccacacattctgacaaattcacagatggtgtatgcctattttggaattgcaatgtcgatagatatcctgctaattccattgtttgtagatttgacactagagtgctatctaaccttaacttgcctggttgtgatggtggcagtttgtatgtaaataaacatgcattccacacaccagcttttgataaaagtgcttttgttaatttaaaacaattaccatttttctattactctgacagtccatgtgagtctcatggaaaacaagtagtgtcagatatagattatgtaccactaaagtctgctacgtgtataacacgttgcaatttaggtggtgctgtctgtagacatcatgctaatgagtacagattgtatctcgatgcttataacatgatgatctcagctggctttagcttgtgggtttacaaacaatttgatacttataacctctggaacacttttacaagacttcagagtttagaaaatgtggcttttaatgttgtaaataagggacactttgatggacaacagggtgaagtaccagtttctatcattaataacactgtttacacaaaagttgatggtgttgatgtagaattgtttgaaaataaaacaacattacctgttaatgtagcatttgagctttgggctaagcgcaacattaaaccagtaccagaggtgaaaatactcaataatttgggtgtggacattgctgctaatactgtgatctgggactacaaaagagatgctccagcacatatatctactattggtgtttgttctatgactgacatagccaagaaaccaactgaaacgatttgtgcaccactcactgtcttttttgatggtagagttgatggtcaagtagacttatttagaaatgcccgtaatggtgttcttattacagaaggtagtgttaaaggtttacaaccatctgtaggtcccaaacaagctagtcttaatggagtcacattaattggagaagccgtaaaaacacagttcaattattataagaaagttgatggtgttgtccaacaattacctgaaacttactttactcagagtagaaatttacaagaatttaaacccaggagtcaaatggaaattgatttcttagaattagctatggatgaattcattgaacggtataaattagaaggctatgccttcgaacatatcgtttatggagattttagtcatagtcagttaggtggtttacatctactgattggactagctaaacgttttaaggaatcaccttttgaattagaagattttattcctatggacagtacagttaaaaactatttcataacagatgcgcaaacaggttcatctaagtgtgtgtgttctgttattgatttattacttgatgattttgttgaaataataaaatcccaagatttatctgtagtttctaaggttgtcaaagtgactattgactatacagaaatttcatttatgctttggtgtaaagatggccatgtagaaacattttacccaaaattacaatctagtcaagcgtggcaaccgggtgttgctatgcctaatctttacaaaatgcaaagaatgctattagaaaagtgtgaccttcaaaattatggtgatagtgcaacattacctaaaggcataatgatgaatgtcgcaaaatatactcaactgtgtcaatatttaaacacattaacattagctgtaccctataatatgagagttatacattttggtgctggttctgataaaggagttgcaccaggtacagctgttttaagacagtggttgcctacgggtacgctgcttgtcgattcagatcttaatgactttgtctctgatgcagattcaactttgattggtgattgtgcaactgtacatacagctaataaatgggatctcattattagtgatatgtacgaccctaagactaaaaatgttacaaaagaaaatgactctaaagagggttttttcacttacatttgtgggtttatacaacaaaagctagctcttggaggttccgtggctataaagataacagaacattcttggaatgctgatctttataagctcatgggacacttcgcatggtggacagcctttgttactaatgtgaatgcgtcatcatctgaagcatttttaattggatgtaattatcttggcaaaccacgcgaacaaatagatggttatgtcatgcatgcaaattacatattttggaggaatacaaatccaattcagttgtcttcctattctttatttgacatgagtaaatttccccttaaattaaggggtactgctgttatgtctttaaaagaaggtcaaatcaatgatatgattttatctcttcttagtaaaggtagacttataattagagaaaacaacagagttgttatttctagtgatgttcttgttaacaactaaacgaacaatgtttgtttttcttgttttattgccactagtctctagtcagtgtgttaatcttacaaccagaactcaattaccccctgcatacactaattctttcacacgtggtgtttattaccctgacaaagttttcagatcctcagttttacattcaactcaggacttgttcttacctttcttttccaatgttacttggttccatgctatacatgtctctgggaccaatggtactaagaggtttgataaccctgtcctaccatttaatgatggtgtttattttgcttccactgagaagtctaacataataagaggctggatttttggtactactttagattcgaagacccagtccctacttattgttaataacgctactaatgttgttattaaagtctgtgaatttcaattttgtaatgatccatttttgggtgtttattaccacaaaaacaacaaaagttggatggaaagtgagttcagagtttattctagtgcgaataattgcacttttgaatatgtctctcagccttttcttatggaccttgaaggaaaacagggtaatttcaaaaatcttagggaatttgtgtttaagaatattgatggttattttaaaatatattctaagcacacgcctattaatttagtgcgtgatctccctcagggtttttcggctttagaaccattggtagatttgccaataggtattaacatcactaggtttcaaactttacttgctttacatagaagttatttgactcctggtgattcttcttcaggttggacagctggtgctgcagcttattatgtgggttatcttcaacctaggacttttctattaaaatataatgaaaatggaaccattacagatgctgtagactgtgcacttgaccctctctcagaaacaaagtgtacgttgaaatccttcactgtagaaaaaggaatctatcaaacttctaactttagagtccaaccaacagaatctattgttagatttcctaatattacaaacttgtgcccttttggtgaagtttttaacgccaccagatttgcatctgtttatgcttggaacaggaagagaatcagcaactgtgttgctgattattctgtcctatataattccgcatcattttccacttttaagtgttatggagtgtctcctactaaattaaatgatctctgctttactaatgtctatgcagattcatttgtaattagaggtgatgaagtcagacaaatcgctccagggcaaactggaaagattgctgattataattataaattaccagatgattttacaggctgcgttatagcttggaattctaacaatcttgattctaaggttggtggtaattataattacctgtatagattgtttaggaagtctaatctcaaaccttttgagagagatatttcaactgaaatctatcaggccggtagcacaccttgtaatggtgttgaaggttttaattgttactttcctttacaatcatatggtttccaacccactaatggtgttggttaccaaccatacagagtagtagtactttcttttgaacttctacatgcaccagcaactgtttgtggacctaaaaagtctactaatttggttaaaaacaaatgtgtcaatttcaacttcaatggtttaacaggcacaggtgttcttactgagtctaacaaaaagtttctgcctttccaacaatttggcagagacattgctgacactactgatgctgtccgtgatccacagacacttgagattcttgacattacaccatgttcttttggtggtgtcagtgttataacaccaggaacaaatacttctaaccaggttgctgttctttatcaggatgttaactgcacagaagtccctgttgctattcatgcagatcaacttactcctacttggcgtgtttattctacaggttctaatgtttttcaaacacgtgcaggctgtttaataggggctgaacatgtcaacaactcatatgagtgtgacatacccattggtgcaggtatatgcgctagttatcagactcagactaattctcctcggcgggcacgtagtgtagctagtcaatccatcattgcctacactatgtcacttggtgcagaaaattcagttgcttactctaataactctattgccatacccacaaattttactattagtgttaccacagaaattctaccagtgtctatgaccaagacatcagtagattgtacaatgtacatttgtggtgattcaactgaatgcagcaatcttttgttgcaatatggcagtttttgtacacaattaaaccgtgctttaactggaatagctgttgaacaagacaaaaacacccaagaagtttttgcacaagtcaaacaaatttacaaaacaccaccaattaaagattttggtggttttaatttttcacaaatattaccagatccatcaaaaccaagcaagaggtcatttattgaagatctacttttcaacaaagtgacacttgcagatgctggcttcatcaaacaatatggtgattgccttggtgatattgctgctagagacctcatttgtgcacaaaagtttaacggccttactgttttgccacctttgctcacagatgaaatgattgctcaatacacttctgcactgttagcgggtacaatcacttctggttggacctttggtgcaggtgctgcattacaaataccatttgctatgcaaatggcttataggtttaatggtattggagttacacagaatgttctctatgagaaccaaaaattgattgccaaccaatttaatagtgctattggcaaaattcaagactcactttcttccacagcaagtgcacttggaaaacttcaagatgtggtcaaccaaaatgcacaagctttaaacacgcttgttaaacaacttagctccaattttggtgcaatttcaagtgttttaaatgatatcctttcacgtcttgacaaagttgaggctgaagtgcaaattgataggttgatcacaggcagacttcaaagtttgcagacatatgtgactcaacaattaattagagctgcagaaatcagagcttctgctaatcttgctgctactaaaatgtcagagtgtgtacttggacaatcaaaaagagttgatttttgtggaaagggctatcatcttatgtccttccctcagtcagcacctcatggtgtagtcttcttgcatgtgacttatgtccctgcacaagaaaagaacttcacaactgctcctgccatttgtcatgatggaaaagcacactttcctcgtgaaggtgtctttgtttcaaatggcacacactggtttgtaacacaaaggaatttttatgaaccacaaatcattactacagacaacacatttgtgtctggtaactgtgatgttgtaataggaattgtcaacaacacagtttatgatcctttgcaacctgaattagactcattcaaggaggagttagataaatattttaagaatcatacatcaccagatgttgatttaggtgacatctctggcattaatgcttcagttgtaaacattcaaaaagaaattgaccgcctcaatgaggttgccaagaatttaaatgaatctctcatcgatctccaagaacttggaaagtatgagcagtatataaaatggccatggtacatttggctaggttttatagctggcttgattgccatagtaatggtgacaattatgctttgctgtatgaccagttgctgtagttgtctcaagggctgttgttcttgtggatcctgctgcaaatttgatgaagacgactctgagccagtgctcaaaggagtcaaattacattacacataaacgaacttatggatttgtttatgagaatcttcacaattggaactgtaactttgaagcaaggtgaaatcaaggatgctactccttcagattttgttcgcgctactgcaacgataccgatacaagcctcactccctttcggatggcttattgttggcgttgcacttcttgctgtttttcagagcgcttccaaaatcataaccctcaaaaagagatggcaactagcactctccaagggtgttcactttgtttgcaacttgctgttgttgtttgtaacagtttactcacaccttttgctcgttgctgctggccttgaagccccttttctctatctttatgctttagtctacttcttgcagagtataaactttgtaagaataataatgaggctttggctttgctggaaatgccgttccaaaaacccattactttatgatgccaactattttctttgctggcatactaattgttacgactattgtataccttacaatagtgtaacttcttcaattgtcattacttcaggtgatggcacaacaagtcctatttctgaacatgactaccagattggtggttatactgaaaaatgggaatctggagtaaaagactgtgttgtattacacagttacttcacttcagactattaccagctgtactcaactcaattgagtacagacactggtgttgaacatgttaccttcttcatctacaataaaattgttgatgagcctgaagaacatgtccaaattcacacaatcgacggttcatccggagttgttaatccagtaatggaaccaatttatgatgaaccgacgacgactactagcgtgcctttgtaagcacaagctgatgagtacgaacttatgtactcattcgtttcggaagagacaggtacgttaatagttaatagcgtacttctttttcttgctttcgtggtattcttgctagttacactagccatccttactgcgcttcgattgtgtgcgtactgctgcaatattgttaacgtgagtcttgtaaaaccttctttttacgtttactctcgtgttaaaaatctgaattcttctagagttcctgatcttctggtctaaacgaactaaatattatattagtttttctgtttggaactttaattttagccatggcagattccaacggtactattaccgttgaagagcttaaaaagctccttgaacaatggaacctagtaataggtttcctattccttacatggatttgtcttctacaatttgcctatgccaacaggaataggtttttgtatataattaagttaattttcctctggctgttatggccagtaactttagcttgttttgtgcttgctgctgtttacagaataaattggatcaccggtggaattgctatcgcaatggcttgtcttgtaggcttgatgtggctcagctacttcattgcttctttcagactgtttgcgcgtacgcgttccatgtggtcattcaatccagaaactaacattcttctcaacgtgccactccatggcactattctgaccagaccgcttctagaaagtgaactcgtaatcggagctgtgatccttcgtggacatcttcgtattgctggacaccatctaggacgctgtgacatcaaggacctgcctaaagaaatcactgttgctacatcacgaacgctttcttattacaaattgggagcttcgcagcgtgtagcaggtgactcaggttttgctgcatacagtcgctacaggattggcaactataaattaaacacagaccattccagtagcagtgacaatattgctttgcttgtacagtaagtgacaacagatgtttcatctcgttgactttcaggttactatagcagagatattactaattattatgaggacttttaaagtttccatttggaatcttgattacatcataaacctcataattaaaaatttatctaagtcactaactgagaataaatattctcaattagatgaagagcaaccaatggagattgattaaacgaacatgaaaattattcttttcttggcactgataacactcgctacttgtgagctttatcactaccaagagtgtgttagaggtacaacagtacttttaaaagaaccttgctcttctggaacatacgagggcaattcaccatttcatcctctagctgataacaaatttgcactgacttgctttagcactcaatttgcttttgcttgtcctgacggcgtaaaacacgtctatcagttacgtgccagatcagtttcacctaaactgttcatcagacaagaggaagttcaagaactttactctccaatttttcttattgttgcggcaatagtgtttataacactttgcttcacactcaaaagaaagacagaatgattgaactttcattaattgacttctatttgtgctttttagcctttctgctattccttgttttaattatgcttattatcttttggttctcacttgaactgcaagatcataatgaaacttgtcacgcctaaacgaacatgaaatttcttgttttcttaggaatcatcacaactgtagctgcatttcaccaagaatgtagtttacagtcatgtactcaacatcaaccatatgtagttgatgacccgtgtcctattcacttctattctaaatggtatattagagtaggagctagaaaatcagcacctttaattgaattgtgcgtggatgaggctggttctaaatcacccattcagtacatcgatatcggtaattatacagtttcctgtttaccttttacaattaattgccaggaacctaaattgggtagtcttgtagtgcgttgttcgttctatgaagactttttagagtatcatgacgttcgtgttgttttagatttcatctaaacgaacaaactaaaatgtctgataatggaccccaaaatcagcgaaatgcaccccgcattacgtttggtggaccctcagattcaactggcagtaaccagaatggagaacgcagtggggcgcgatcaaaacaacgtcggccccaaggtttacccaataatactgcgtcttggttcaccgctctcactcaacatggcaaggaagaccttaaattccctcgaggacaaggcgttccaattaacaccaatagcagtccagatgaccaaattggctactaccgaagagctaccagacgaattcgtggtggtgacggtaaaatgaaagatctcagtccaagatggtatttctactacctaggaactgggccagaagctggacttccctatggtgctaacaaagacggcatcatatgggttgcaactgagggagccttgaatacaccaaaagatcacattggcacccgcaatcctgctaacaatgctgcaatcgtgctacaacttcctcaaggaacaacattgccaaaaggcttctacgcagaagggagcagaggcggcagtcaagcctcttctcgttcctcatcacgtagtcgcaacagttcaagaaattcaactccaggcagcagtaggggaacttctcctgctagaatggctggcaatggcggtgatgctgctcttgctttgctgctgcttgacagattgaaccagcttgagagcaaaatgtctggtaaaggccaacaacaacaaggccaaactgtcactaagaaatctgctgctgaggcttctaagaagcctcggcaaaaacgtactgccactaaagcatacaatgtaacacaagctttcggcagacgtggtccagaacaaacccaaggaaattttggggaccaggaactaatcagacaaggaactgattacaaacattggccgcaaattgcacaatttgcccccagcgcttcagcgttcttcggaatgtcgcgcattggcatggaagtcacaccttcgggaacgtggttgacctacacaggtgccatcaaattggatgacaaagatccaaatttcaaagatcaagtcattttgctgaataagcatattgacgcatacaaaacattcccaccaacagagcctaaaaaggacaaaaagaagaaggctgatgaaactcaagccttaccgcagagacagaagaaacagcaaactgtgactcttcttcctgctgcagatttggatgatttctccaaacaattgcaacaatccatgagcagtgctgactcaactcaggcctaaactcatgcagaccacacaaggcagatgggctatataaacgttttcgcttttccgtttacgatatatagtctactcttgtgcagaatgaattctcgtaactacatagcacaagtagatgtagttaactttaatctcacatagcaatctttaatcagtgtgtaacattagggaggacttgaaagagccaccacattttcaccgaggccacgcggagtacgatcgagtgtacagtgaacaatgctagggagagctgcctatatggaagagccctaatgtgtaaaattaattttagtagtgctatccccatgtgattttaatagcttcttaggagaatgacaaaaaaaaaaaaaaaaaaaaaaaaaaaaaaaaa

SEQ ID NO: 164 - protein, 7096 aa, betacoronavirus SARS coronavirus 2 [sequence omitted]

SEQ ID NO: 165 - protein, 1273 aa, betacoronavirus SARS coronavirus 2
MFVFLVLLPLVSSQCVNLTTRTQLPPAYTNSFTRGVYYPDKVFRSSVLHSTQDLFLPFFSNVTWFHAIHVSGTNGTKRFDNPVLPFNDGVYFASTEKSNIIRGWIFGTTLDSKTQSLLIVNNATNVVIKVCEFQFCNDPFLGVYYHKNNKSWMESEFRVYSSANNCTFEYVSQPFLMDLEGKQGNFKNLREFVFKNIDGYFKIYSKHTPINLVRDLPQGFSALEPLVDLPIGINITRFQTLLALHRSYLTPGDSSSGWTAGAAAYYVGYLQPRTFLLKYNENGTITDAVDCALDPLSETKCTLKSFTVEKGIYQTSNFRVQPTESIVRFPNITNLCPFGEVFNATRFASVYAWNRKRISNCVADYSVLYNSASFSTFKCYGVSPTKLNDLCFTNVYADSFVIRGDEVRQIAPGQTGKIADYNYKLPDDFTGCVIAWNSNNLDSKVGGNYNYLYRLFRKSNLKPFERDISTEIYQAGSTPCNGVEGFNCYFPLQSYGFQPTNGVGYQPYRVVVLSFELLHAPATVCGPKKSTNLVKNKCVNFNFNGLTGTGVLTESNKKFLPFQQFGRDIADTTDAVRDPQTLEILDITPCSFGGVSVITPGTNTSNQVAVLYQDVNCTEVPVAIHADQLTPTWRVYSTGSNVFQTRAGCLIGAEHVNNSYECDIPIGAGICASYQTQTNSPRRARSVASQSIIAYTMSLGAENSVAYSNNSIAIPTNFTISVTTEILPVSMTKTSVDCTMYICGDSTECSNLLLQYGSFCTQLNRALTGIAVEQDKNTQEVFAQVKQIYKTPPIKDFGGFNFSQILPDPSKPSKRSFIEDLLFNKVTLADAGFIKQYGDCLGDIAARDLICAQKFNGLTVLPPLLTDEMIAQYTSALLAGTITSGWTFGAGAALQIPFAMQMAYRFNGIGVTQNVLYENQKLIANQFNSAIGKIQDSLSSTASALGKLQDVVNQNAQALNTLVKQLSSNFGAISSVLNDILSRLDKVEAEVQIDRLITGRLQSLQTYVTQQLIRAAEIRASANLAATKMSECVLGQSKRVDFCGKGYHLMSFPQSAPHGVVFLHVTYVPAQEKNFTTAPAICHDGKAHFPREGVFVSNGTHWFVTQRNFYEPQIITTDNTFVSGNCDVVIGIVNNTVYDPLQPELDSFKEELDKYFKNHTSPDVDLGDISGINASVVNIQKEIDRLNEVAKNLNESLIDLQELGKYEQYIKWPWYIWLGFIAGLIAIVMVTIMLCCMTSCCSCLKGCCSCGSCCKFDEDDSEPVLKGVKLHYT

SEQ ID NO: 166 - protein, 220 aa, synthetic construct
  REGION 1..220: note = surface glycoprotein RBD [Wuhan seafood market pneumonia virus]
NITNLCPFGEVFNATRFASVYAWNRKRISNCVADYSVLYNSASFSTFKCYGVSPTKLNDLCFTNVYADSFVIRGDEVRQIAPGQTGKIADYNYKLPDDFTGCVIAWNSNNLDSKVGGNYNYLYRLFRKSNLKPFERDISTEIYQAGSTPCNGVEGFNCYFPLQSYGFQPTNGVGYQPYRVVVLSFELLHAPATVCGPKKSTNLVKNKCVNFNFNGLTGTG

SEQ ID NO: 167 - protein, 72 aa, synthetic construct
  REGION 1..72: note = Receptor Binding Motif (RBM) in surface glycoprotein RBD [Wuhan seafood market pneumonia virus]
NSNNLDSKVGGNYNYLYRLFRKSNLKPFERDISTEIYQAGSTPCNGVEGFNCYFPLQSYGFQPTNGVGYQPY

SEQ ID NO: 168 - protein, 107 aa, synthetic construct [sequence omitted]

SEQ ID NO: 169 - protein, 7 aa, synthetic construct
  REGION 1..7: note = SARS-CoV-2 S309-v13 mAb CDRL1
QTVSSTS

SEQ ID NO: 170 - skipped

SEQ ID NO: 171 - protein, 8 aa, synthetic construct
  REGION 1..8: note = SARS-CoV-2 S309-v13 mAb CDRL3
QQHDTSLT

SEQ ID NO: 172 - protein, 127 aa, synthetic construct
  REGION 1..127: note = SARS-CoV-2 S309-v2.9 mAb VH
QVQLVQSGAEVKKPGASVKVSCKASGYPFTSYGISWVRQAPGQGLEWMGFISTYNANTNYAQKFQGRVTMTTDTSTTTGYMELRRLRSDDTAVYYCARDYTRGAFFGESLIGGFDNWGQGTLVTVSS

SEQ ID NO: 173 - protein, 330 aa, synthetic construct
  REGION 1..330: note = SARS-CoV-2 CH1-CH3 G1m17; IgG1*01 LS
ASTKGPSVFPLAPSSKSTSGGTAALGCLVKDYFPEPVTVSWNSGALTSGVHTFPAVLQSSGLYSLSSVVTVPSSSLGTQTYICNVNHKPSNTKVDKKVEPKSCDKTHTCPPCPAPELLGGPSVFLFPPKPKDTLMISRTPEVTCVVVDVSHEDPEVKFNWYVDGVEVHNAKTKPREEQYNSTYRVVSVLTVLHQDWLNGKEYKCKVSNKALPAPIEKTISKAKGQPREPQVYTLPPSRDELTKNQVSLTCLVKGFYPSDIAVEWESNGQPENNYKTTPPVLDSDGSFFLYSKLTVDKSRWQQGNVFSCSVLHEALHSHYTQKSLSLSPGK

SEQ ID NO: 174 - protein, 107 aa, synthetic construct [sequence omitted]

SEQ ID NO: 175 - protein, 330 aa, synthetic construct
  REGION 1..330: note = SARS-CoV-2 CH1-CH3 G1m17; IgG1*01 LS GAALIE
ASTKGPSVFPLAPSSKSTSGGTAALGCLVKDYFPEPVTVSWNSGALTSGVHTFPAVLQSSGLYSLSSVVTVPSSSLGTQTYICNVNHKPSNTKVDKKVEPKSCDKTHTCPPCPAPELLAGPSVFLFPPKPKDTLMISRTPEVTCVVVDVSHEDPEVKFNWYVDGVEVHNAKTKPREEQYNSTYRVVSVLTVLHQDWLNGKEYKCKVSNKALPLPEEKTISKAKGQPREPQVYTLPPSRDELTKNQVSLTCLVKGFYPSDIAVEWESNGQPENNYKTTPPVLDSDGSFFLYSKLTVDKSRWQQGNVFSCSVLHEALHSHYTQKSLSLSPGK

SEQ ID NO: 176 - protein, 123 aa, synthetic construct
  REGION 1..123: note = SARS-CoV-2 S300-v2.10 mAb VH
QVQLVQSGAEVKKPGASVKVSCKASGYTFTDYYIHWVRQAPGQGPEWLGFVNAYSGATRYAQKYQGRVTMTRDTSISTAYMQLSRLRPDDTAVYYCARDRPSHEFAMYFFDNWGQGTLVTVSS

SEQ ID NO: 177 - protein, 123 aa, synthetic construct
  REGION 1..123: note = SARS-CoV-2 S300-v2.11 mAb VH
QVQLVQSGAEVKKPGASVKVSCKASGYTFTDYYIHWVRQAPGQGPEWLGFVQGYSGATRYAQKYQGRVTMTRDTSISTAYMQLSRLRPDDTAVYYCARDRPSHEFAMYFFDNWGQGTLVTVSS

SEQ ID NO: 178 - protein, 124 aa, synthetic construct
  REGION 1..124: note = SARS-CoV-2 S315-v1 mAb VH
EVQLVESGGGLVQPGGSLRLSCAASGFTFSNYWMTWVRQAPGKGLEWVANIKQDGSEKYYVDSVKGRFTISRDNAKNSLYLQMNSLRAEDTAVYYCARDLWWNDQAHYYGMDVWGQGTTVTVSS

SEQ ID NO: 179 - protein, 8 aa, synthetic construct
  REGION 1..8: note = SARS-CoV-2 S315-v1 mAb CDRH1
GFTFSNYW

SEQ ID NO: 180 - protein, 8 aa, synthetic construct
  REGION 1..8: note = SARS-CoV-2 S315-v1 mAb CDRH2
IKQDGSEK

SEQ ID NO: 181 - protein, 17 aa, synthetic construct
  REGION 1..17: note = SARS-CoV-2 S315-v1 mAb CDRH3
ARDLWWNDQAHYYGMDV

SEQ ID NO: 182 - protein, 106 aa, synthetic construct
  REGION 1..106: note = SARS-CoV-2 S315-v1 mAb VL
SYELTQPPSVSVSPGQTARITCSGDAFPNQYAYWYQQKPGQAPVMLIYKDSERPSGIPERFFGSSSGTTVTLTIRGVQAEDEADYYCQSADSSGTVFGGGTKLTVL

SEQ ID NO: 183 - protein, 6 aa, synthetic construct
  REGION 1..6: note = SARS-CoV-2 S315-v1 mAb CDRL1
AFPNQY

SEQ ID NO: 184 - skipped

SEQ ID NO: 185 - protein, 9 aa, synthetic construct
  REGION 1..9: note = SARS-CoV-2 S315-v1 mAb CDRL3
QSADSSGTV

SEQ ID NO: 186 - DNA, 373 bp, synthetic construct
  misc_feature 1..373: note = SARS-CoV-2 S315-v1 mAb VH
  source 1..373: mol_type = other DNA
gaggtgcagctggtggagtctgggggaggcttggtccagcctggggggtccctgagactctcctgtgcagcctctggattcacctttagtaattattggatgacctgggtccgccaggctccagggaaggggctggagtgggtggccaacataaagcaagatggaagtgagaaatactatgtggactctgtgaagggccgattcaccatctccagagacaacgccaagaactcactgtatctgcaaatgaacagcctgagagccgaggacacggctgtgtattactgtgcgagagatctttggtggaacgaccaggctcactactacggtatggacgtctggggccaagggaccacggtcaccgtctcctcag

SEQ ID NO: 187 - DNA, 319 bp, synthetic construct
  misc_feature 1..319: note = SARS-CoV-2 S315-v1 mAb VL
  source 1..319: mol_type = other DNA
tcctatgagctgacacagccaccctcggtgtcagtgtccccaggacagacggccaggatcacctgctctggagatgcattcccaaaccaatatgcttattggtaccagcagaagccaggccaggcccctgtgatgctgatctataaagacagtgagaggccctcagggatccctgagcgattctttggctccagctcagggacaacagtcacgttgaccatcagaggagtccaggcagaagacgaggctgactattactgtcaatcagcagacagcagtggtaccgtgttcggcggagggaccaagctgaccgtcctag

SEQ ID NO: 188 - DNA, 372 bp, synthetic construct
  misc_feature 1..372: note = SARS-CoV-2 S315-v1 mAb VH (nt - codon optimized)
  source 1..372: mol_type = other DNA
gaagtgcagcttgtcgagagcggcggaggcctcgttcagccaggtgggagtctccgtctttcatgcgccgcttcaggatttacgttctccaactactggatgacatgggtgaggcaggcacctgggaaggggctggagtgggtggctaacatcaagcaggacggatctgaaaaatattatgtagattctgtgaaggggcggtttaccatctcaagggataatgccaaaaactctttgtatttacagatgaactctcttcgagccgaggacaccgccgtttactactgtgcccgagatctatggtggaatgaccaggctcactattatggaatggacgtgtggggccagggtactaccgttaccgtctcctca

SEQ ID NO: 189 - DNA, 318 bp, synthetic construct
  misc_feature 1..318: note = SARS-CoV-2 S315-v1 mAb VL (nt- codon optimized)
  source 1..318: mol_type = other DNA
tcttacgagctcacccagccaccctcagtgtcagtgagccctggccaaacagctcgcatcacctgttcaggtgacgcctttccaaatcagtacgcctactggtatcagcagaaacccggccaggcacccgttatgctcatctacaaagattctgagcggccatccggtatccccgaacgctttttcggaagctccagtgggactacagttacacttactatccggggagtgcaagctgaagatgaggccgactattattgccagagcgcagactcctcaggcacagtgtttgggggcgggactaaactaactgtgctg

SEQ ID NO: 190 - protein, 106 aa, synthetic construct
  REGION 1..106: note = SARS-CoV-2 S315-v2 mAb VL
SYELTQPPSVSVSPGQTARITCSGDAFPNQYAYWYQQKPGQAPVMLIYKDSERPSGIPERFFGSSSGTTVTLTISGVQAEDEADYYCQSADSSGTVFGGGTKLTVL

SEQ ID NO: 191 - DNA, 319 bp, synthetic construct
  misc_feature 1..319: note = SARS-CoV-2 S315-v2 mAb VL
  source 1..319: mol_type = other DNA
tcctatgagctgacacagccaccctcggtgtcagtgtccccaggacagacggccaggatcacctgctctggagatgcattcccaaaccaatatgcttattggtaccagcagaagccaggccaggcccctgtgatgctgatctataaagacagtgagaggccctcagggatccctgagcgattctttggctccagctcagggacaacagtcacgttgaccatcagtggagtccaggcagaagacgaggctgactattactgtcaatcagcagacagcagtggtaccgtgttcggcggagggaccaagctgaccgtcctag

SEQ ID NO: 192 - DNA, 318 bp, synthetic construct
  misc_feature 1..318: note = SARS-CoV-2 S315-v2 mAb VL (nt - codon optimized)
  source 1..318: mol_type = other DNA
tcctacgagctcacccagcccccctcagtctctgtgtctcctggacagacagccagaatcacctgctcgggagatgcttttcccaaccaatacgcctactggtaccaacagaaaccaggtcaggcgcctgtcatgctgatttataaagactcagagcggccttcaggaattcccgaaagattcttcgggagttcaagcggaactaccgtgaccttaaccataagcggggtgcaggccgaagatgaagcagactattattgccagagtgccgatagtagtggcacagtctttgggggggggacaaagctgacagtactc

SEQ ID NO: 193 - protein, 106 aa, synthetic construct
  REGION 1..106: note = SARS-CoV-2 mAb CL IgLC*01
GQPKAAPSVTLFPPSSEELQANKATLVCLISDFYPGAVTVAWKADSSPVKAGVETTTPSKQSNNKYAASSYLSLTPEQWKSHRSYSCQVTHEGSTVEKTVAPTECS

SEQ ID NO: 194 - protein, 124 aa, synthetic construct
  REGION 1..124: note = SARS-CoV-2 S315-v3 mAb VH
EVQLVESGGGLVQPGGSLRLSCAASGFTFSNYFMTWVRQAPGKGLEWVANIKQDGSEKYYVDSVKGRFTISRDNAKNSLYLQMNSLRAEDTAVYYCARDLWWNDQAHYYGMDVWGQGTTVTVSS

SEQ ID NO: 195 - protein, 8 aa, synthetic construct
  REGION 1..8: note = SARS-CoV-2 S315-v3 mAb CDRH1
GFTFSNYF

SEQ ID NO: 196 - protein, 124 aa, synthetic construct
  REGION 1..124: note = SARS-CoV-2 S315-v4 mAb VH
EVQLVESGGGLVQPGGSLRLSCAASGFTFSNYWMTWVRQAPGKGLEWVANIKQDASEKYYVDSVKGRFTISRDNAKNSLYLQMNSLRAEDTAVYYCARDLWWNDQAHYYGMDVWGQGTTVTVSS

SEQ ID NO: 197 - protein, 8 aa, synthetic construct
  REGION 1..8: note = SARS-CoV-2 S315-v4 mAb CDRH2
IKQDASEK

SEQ ID NO: 198 - protein, 124 aa, synthetic construct
  REGION 1..124: note = SARS-CoV-2 S315-v5 mAb VH
EVQLVESGGGLVQPGGSLRLSCAASGFTFSNYWMTWVRQAPGKGLEWVANIKQEGSEKYYVDSVKGRFTISRDNAKNSLYLQMNSLRAEDTAVYYCARDLWWNDQAHYYGMDVWGQGTTVTVSS

SEQ ID NO: 199 - protein, 8 aa, synthetic construct
  REGION 1..8: note = SARS-CoV-2 S315-v5 mAb CDRH2
IKQEGSEK

SEQ ID NO: 200 - protein, 124 aa, synthetic construct
  REGION 1..124: note = SARS-CoV-2 S315-v6 mAb VH
EVQLVESGGGLVQPGGSLRLSCAASGFTFSNYWMTWVRQAPGKGLEWVANIKQDGSEKYYVDSVKGRFTISRDNAKNSLYLQMNSLRAEDTAVYYCARDLFWNDQAHYYGMDVWGQGTTVTVSS

SEQ ID NO: 201 - protein, 17 aa, synthetic construct
  REGION 1..17: note = SARS-CoV-2 S315-v6 mAb CDRH3
ARDLFWNDQAHYYGMDV

SEQ ID NO: 202 - protein, 124 aa, synthetic construct
  REGION 1..124: note = SARS-CoV-2 S315-v7 mAb VH
EVQLVESGGGLVQPGGSLRLSCAASGFTFSNYWMTWVRQAPGKGLEWVANIKQDGSEKYYVDSVKGRFTISRDNAKNSLYLQMNSLRAEDTAVYYCARDLWFNDQAHYYGMDVWGQGTTVTVSS

SEQ ID NO: 203 - protein, 17 aa, synthetic construct
  REGION 1..17: note = SARS-CoV-2 S315-v7 mAb CDRH3
ARDLWFNDQAHYYGMDV

SEQ ID NO: 204 - protein, 230 aa, synthetic construct
  REGION 1..230: note = SARS-CoV-2 Heavy Chain IgHG1*01 Fd
QVQLVQSGAEVKKPGASVKVSCKASGYPFTSYGISWVRQAPGQGLEWMGWISTYNGNTNYAQKFQGRVTMTTDTSTTTGYMELRRLRSDDTAVYYCARDYTRGAWFGESLIGGFDNWGQGTLVTVSSASTKGPSVFPLAPSSKSTSGGTAALGCLVKDYFPEPVTVSWNSGALTSGVHTFPAVLQSSGLYSLSSVVTVPSSSLGTQTYICNVNHKPSNTKVDKRVEPKSC

SEQ ID NO: 205 - protein, 214 aa, synthetic construct
  REGION 1..214: note = SARS-CoV-2 Light Chain IgKC*01
EIVLTQSPGTLSLSPGERATLSCRASQTVSSTSLAWYQQKPGQAPRLLIYGASSRATGIPDRFSGSGSGTDFTLTISRLEPEDFAVYYCQQHDTSLTFGGGTKVEIKRTVAAPSVFIFPPSDEQLKSGTASVVCLLNNFYPREAKVQWKVDNALQSGNSQESVTEQDSKDSTYSLSSTLTLSKADYEKHKVYACEVTHQGLSSPVTKSFNRGEC

SEQ ID NO: 206 - protein, 18 aa, synthetic construct
  REGION 1..18: note = Linker
GSTSGSGKPGSGEGSTKG

SEQ ID NO: 207 - protein, 10 aa, synthetic construct
  REGION 1..10: note = Linker
GSGKPGSGEG

SEQ ID NO: 208 - protein, 8 aa, synthetic construct
  REGION 1..8: note = Linker
GKPGSGEG

SEQ ID NO: 209 - protein, 8 aa, synthetic construct
  REGION 1..8: note = Linker
SGKPGSGE

SEQ ID NO: 210 - skipped

SEQ ID NO: 211 - protein, 121 aa, synthetic construct
  REGION 1..121: note = Linker
  VARIANT 2..10: note = any one or all of amino acids 2-10 can either be present or absent
  VARIANT 12..121: note = any one or all of amino acids 12-121 can either be present or absent
GGGGGGGGGGSGGGGGGGGGGSGGGGGGGGGGSGGGGGGGGGGSGGGGGGGGGGSGGGGGGGGGGSGGGGGGGGGGSGGGGGGGGGGSGGGGGGGGGGSGGGGGGGGGGSGGGGGGGGGGS

SEQ ID NO: 212 - protein, 15 aa, synthetic construct
  REGION 1..15: note = Linker
GGGGSGGGGSGGGGS

SEQ ID NO: 213 - protein, 50 aa, synthetic construct
  REGION 1..50: note = Linker
GGGGSGGGGSGGGGSGGGGSGGGGSGGGGSGGGGSGGGGSGGGGSGGGGS

SEQ ID NO: 214 - protein, 18 aa, synthetic construct
  REGION 1..18: note = Linker
GSTSGGGSGGGSGGGGSS

SEQ ID NO: 215 - protein, 14 aa, synthetic construct
  REGION 1..14: note = Linker
EGKSSGSGSESKVD

SEQ ID NO: 216 - protein, 18 aa, synthetic construct
  REGION 1..18: note = Linker
KESGSVSSEQLAQFRSLD

SEQ ID NO: 217 - protein, 5 aa, synthetic construct
  REGION 1..5: note = Linker
GGGGS

SEQ ID NO: 218 - protein, 494 aa, synthetic construct
  REGION 1..494: note = SARS-CoV-2 Synthetic sequence S309-scFab (H-L)
QVQLVQSGAEVKKPGASVKVSCKASGYPFTSYGISWVRQAPGQGLEWMGWISTYNGNTNYAQKFQGRVTMTTDTSTTTGYMELRRLRSDDTAVYYCARDYTRGAWFGESLIGGFDNWGQGTLVTVSSASTKGPSVFPLAPSSKSTSGGTAALGCLVKDYFPEPVTVSWNSGALTSGVHTFPAVLQSSGLYSLSSVVTVPSSSLGTQTYICNVNHKPSNTKVDKRVEPKSCGGGGSGGGGSGGGGSGGGGSGGGGSGGGGSGGGGSGGGGSGGGGSGGGGSEIVLTQSPGTLSLSPGERATLSCRASQTVSSTSLAWYQQKPGQAPRLLIYGASSRATGIPDRFSGSGSGTDFTLTISRLEPEDFAVYYCQQHDTSLTFGGGTKVEIKRTVAAPSVFIFPPSDEQLKSGTASVVCLLNNFYPREAKVQWKVDNALQSGNSQESVTEQDSKDSTYSLSSTLTLSKADYEKHKVYACEVTHQGLSSPVTKSFNRGEC

SEQ ID NO: 219 - protein, 494 aa, synthetic construct
  REGION 1..494: note = SARS-CoV-2 S309-scFab (L-H)
EIVLTQSPGTLSLSPGERATLSCRASQTVSSTSLAWYQQKPGQAPRLLIYGASSRATGIPDRFSGSGSGTDFTLTISRLEPEDFAVYYCQQHDTSLTFGGGTKVEIKRTVAAPSVFIFPPSDEQLKSGTASVVCLLNNFYPREAKVQWKVDNALQSGNSQESVTEQDSKDSTYSLSSTLTLSKADYEKHKVYACEVTHQGLSSPVTKSFNRGECGGGGSGGGGSGGGGSGGGGSGGGGSGGGGSGGGGSGGGGSGGGGSGGGGSQVQLVQSGAEVKKPGASVKVSCKASGYPFTSYGISWVRQAPGQGLEWMGWISTYNGNTNYAQKFQGRVTMTTDTSTTTGYMELRRLRSDDTAVYYCARDYTRGAWFGESLIGGFDNWGQGTLVTVSSASTKGPSVFPLAPSSKSTSGGTAALGCLVKDYFPEPVTVSWNSGALTSGVHTFPAVLQSSGLYSLSSVVTVPSSSLGTQTYICNVNHKPSNTKVDKRVEPKSC

SEQ ID NO: 220 - protein, 249 aa, synthetic construct
  REGION 1..249: note = SARS-CoV-2 S309-scFv (VH-VL)
QVQLVQSGAEVKKPGASVKVSCKASGYPFTSYGISWVRQAPGQGLEWMGWISTYNGNTNYAQKFQGRVTMTTDTSTTTGYMELRRLRSDDTAVYYCARDYTRGAWFGESLIGGFDNWGQGTLVTVSSGGGGSGGGGSGGGGSEIVLTQSPGTLSLSPGERATLSCRASQTVSSTSLAWYQQKPGQAPRLLIYGASSRATGIPDRFSGSGSGTDFTLTISRLEPEDFAVYYCQQHDTSLTFGGGTKVEIK

SEQ ID NO: 221 - protein, 249 aa, synthetic construct
  REGION 1..249: note = SARS-CoV-2 S309-scFv (VL-VH)
EIVLTQSPGTLSLSPGERATLSCRASQTVSSTSLAWYQQKPGQAPRLLIYGASSRATGIPDRFSGSGSGTDFTLTISRLEPEDFAVYYCQQHDTSLTFGGGTKVEIKGGGGSGGGGSGGGGSQVQLVQSGAEVKKPGASVKVSCKASGYPFTSYGISWVRQAPGQGLEWMGWISTYNGNTNYAQKFQGRVTMTTDTSTTTGYMELRRLRSDDTAVYYCARDYTRGAWFGESLIGGFDNWGQGTLVTVSS

SEQ ID NO: 222 - protein, 518 aa, synthetic construct
  REGION 1..518: note = SARS-CoV-2 S309-scFv (VH-VL)-(VH-VL)
QVQLVQSGAEVKKPGASVKVSCKASGYPFTSYGISWVRQAPGQGLEWMGWISTYNGNTNYAQKFQGRVTMTTDTSTTTGYMELRRLRSDDTAVYYCARDYTRGAWFGESLIGGFDNWGQGTLVTVSSGGGGSGGGGSGGGGSEIVLTQSPGTLSLSPGERATLSCRASQTVSSTSLAWYQQKPGQAPRLLIYGASSRATGIPDRFSGSGSGTDFTLTISRLEPEDFAVYYCQQHDTSLTFGGGTKVEIKGGGGSGGGGSGGGGSGGGGSQVQLVQSGAEVKKPGASVKVSCKASGYPFTSYGISWVRQAPGQGLEWMGWISTYNGNTNYAQKFQGRVTMTTDTSTTTGYMELRRLRSDDTAVYYCARDYTRGAWFGESLIGGFDNWGQGTLVTVSSGGGGSGGGGSGGGGSEIVLTQSPGTLSLSPGERATLSCRASQTVSSTSLAWYQQKPGQAPRLLIYGASSRATGIPDRFSGSGSGTDFTLTISRLEPEDFAVYYCQQHDTSLTFGGGTKVEIK

SEQ ID NO: 223 - protein, 518 aa, synthetic construct
  REGION 1..518: note = SARS-CoV-2 S309-scFv-(VH-VL)-(VL-VH)
QVQLVQSGAEVKKPGASVKVSCKASGYPFTSYGISWVRQAPGQGLEWMGWISTYNGNTNYAQKFQGRVTMTTDTSTTTGYMELRRLRSDDTAVYYCARDYTRGAWFGESLIGGFDNWGQGTLVTVSSGGGGSGGGGSGGGGSEIVLTQSPGTLSLSPGERATLSCRASQTVSSTSLAWYQQKPGQAPRLLIYGASSRATGIPDRFSGSGSGTDFTLTISRLEPEDFAVYYCQQHDTSLTFGGGTKVEIKGGGGSGGGGSGGGGSGGGGSEIVLTQSPGTLSLSPGERATLSCRASQTVSSTSLAWYQQKPGQAPRLLIYGASSRATGIPDRFSGSGSGTDFTLTISRLEPEDFAVYYCQQHDTSLTFGGGTKVEIKGGGGSGGGGSGGGGSQVQLVQSGAEVKKPGASVKVSCKASGYPFTSYGISWVRQAPGQGLEWMGWISTYNGNTNYAQKFQGRVTMTTDTSTTTGYMELRRLRSDDTAVYYCARDYTRGAWFGESLIGGFDNWGQGTLVTVSS

SEQ ID NO: 224 - protein, 518 aa, synthetic construct
  REGION 1..518: note = SARS-CoV-2 S309-scFv-(VL-VH)-(VH-VL)
EIVLTQSPGTLSLSPGERATLSCRASQTVSSTSLAWYQQKPGQAPRLLIYGASSRATGIPDRFSGSGSGTDFTLTISRLEPEDFAVYYCQQHDTSLTFGGGTKVEIKGGGGSGGGGSGGGGSQVQLVQSGAEVKKPGASVKVSCKASGYPFTSYGISWVRQAPGQGLEWMGWISTYNGNTNYAQKFQGRVTMTTDTSTTTGYMELRRLRSDDTAVYYCARDYTRGAWFGESLIGGFDNWGQGTLVTVSSGGGGSGGGGSGGGGSGGGGSQVQLVQSGAEVKKPGASVKVSCKASGYPFTSYGISWVRQAPGQGLEWMGWISTYNGNTNYAQKFQGRVTMTTDTSTTTGYMELRRLRSDDTAVYYCARDYTRGAWFGESLIGGFDNWGQGTLVTVSSGGGGSGGGGSGGGGSEIVLTQSPGTLSLSPGERATLSCRASQTVSSTSLAWYQQKPGQAPRLLIYGASSRATGIPDRFSGSGSGTDFTLTISRLEPEDFAVYYCQQHDTSLTFGGGTKVEIK

SEQ ID NO: 225 - protein, 518 aa, synthetic construct
  REGION 1..518: note = Synthetic sequence SARS-CoV-2 S309-scFv-(VL-VH)-(VL-VH)
EIVLTQSPGTLSLSPGERATLSCRASQTVSSTSLAWYQQKPGQAPRLLIYGASSRATGIPDRFSGSGSGTDFTLTISRLEPEDFAVYYCQQHDTSLTFGGGTKVEIKGGGGSGGGGSGGGGSQVQLVQSGAEVKKPGASVKVSCKASGYPFTSYGISWVRQAPGQGLEWMGWISTYNGNTNYAQKFQGRVTMTTDTSTTTGYMELRRLRSDDTAVYYCARDYTRGAWFGESLIGGFDNWGQGTLVTVSSGGGGSGGGGSGGGGSGGGGSEIVLTQSPGTLSLSPGERATLSCRASQTVSSTSLAWYQQKPGQAPRLLIYGASSRATGIPDRFSGSGSGTDFTLTISRLEPEDFAVYYCQQHDTSLTFGGGTKVEIKGGGGSGGGGSGGGGSQVQLVQSGAEVKKPGASVKVSCKASGYPFTSYGISWVRQAPGQGLEWMGWISTYNGNTNYAQKFQGRVTMTTDTSTTTGYMELRRLRSDDTAVYYCARDYTRGAWFGESLIGGFDNWGQGTLVTVSS

SEQ ID NO: 226 - protein, 494 aa, synthetic construct
  REGION 1..494: note = Synthetic sequence SARS-CoV-2 S309-scFab-(H-L) v1.1
QVQLVQSGAEVKKPGASVKVSCKASGYPFTSYGISWVRQAPGQGLEWMGWISTYQGNTNYAQKFQGRVTMTTDTSTTTGYMELRRLRSDDTAVYYCARDYTRGAWFGESLIGGFDNWGQGTLVTVSSASTKGPSVFPLAPSSKSTSGGTAALGCLVKDYFPEPVTVSWNSGALTSGVHTFPAVLQSSGLYSLSSVVTVPSSSLGTQTYICNVNHKPSNTKVDKRVEPKSCGGGGSGGGGSGGGGSGGGGSGGGGSGGGGSGGGGSGGGGSGGGGSGGGGSEIVLTQSPGTLSLSPGERATLSCRASQTVSSTSLAWYQQKPGQAPRLLIYGASSRATGIPDRFSGSGSGTDFTLTISRLEPEDFAVYYCQQHDTSLTFGGGTKVEIKRTVAAPSVFIFPPSDEQLKSGTASVVCLLNNFYPREAKVQWKVDNALQSGNSQESVTEQDSKDSTYSLSSTLTLSKADYEKHKVYACEVTHQGLSSPVTKSFNRGEC

SEQ ID NO: 227 - protein, 494 aa, synthetic construct
  REGION 1..494: note = Synthetic sequence SARS-CoV-2 S309-scFab-(L-H) v1.1
EIVLTQSPGTLSLSPGERATLSCRASQTVSSTSLAWYQQKPGQAPRLLIYGASSRATGIPDRFSGSGSGTDFTLTISRLEPEDFAVYYCQQHDTSLTFGGGTKVEIKRTVAAPSVFIFPPSDEQLKSGTASVVCLLNNFYPREAKVQWKVDNALQSGNSQESVTEQDSKDSTYSLSSTLTLSKADYEKHKVYACEVTHQGLSSPVTKSFNRGECGGGGSGGGGSGGGGSGGGGSGGGGSGGGGSGGGGSGGGGSGGGGSGGGGSQVQLVQSGAEVKKPGASVKVSCKASGYPFTSYGISWVRQAPGQGLEWMGWISTYQGNTNYAQKFQGRVTMTTDTSTTTGYMELRRLRSDDTAVYYCARDYTRGAWFGESLIGGFDNWGQGTLVTVSSASTKGPSVFPLAPSSKSTSGGTAALGCLVKDYFPEPVTVSWNSGALTSGVHTFPAVLQSSGLYSLSSVVTVPSSSLGTQTYICNVNHKPSNTKVDKRVEPKSC

SEQ ID NO: 228 - protein, 249 aa, synthetic construct
  REGION 1..249: note = Synthetic sequence SARS-CoV-2 S309-scFv-(VH-VL) v1.1
QVQLVQSGAEVKKPGASVKVSCKASGYPFTSYGISWVRQAPGQGLEWMGWISTYQGNTNYAQKFQGRVTMTTDTSTTTGYMELRRLRSDDTAVYYCARDYTRGAWFGESLIGGFDNWGQGTLVTVSSGGGGSGGGGSGGGGSEIVLTQSPGTLSLSPGERATLSCRASQTVSSTSLAWYQQKPGQAPRLLIYGASSRATGIPDRFSGSGSGTDFTLTISRLEPEDFAVYYCQQHDTSLTFGGGTKVEIK

SEQ ID NO: 229 - protein, 249 aa, synthetic construct
  REGION 1..249: note = Synthetic sequence SARS-CoV-2 S309-scFv-(VL-VH) v1.1
EIVLTQSPGTLSLSPGERATLSCRASQTVSSTSLAWYQQKPGQAPRLLIYGASSRATGIPDRFSGSGSGTDFTLTISRLEPEDFAVYYCQQHDTSLTFGGGTKVEIKGGGGSGGGGSGGGGSQVQLVQSGAEVKKPGASVKVSCKASGYPFTSYGISWVRQAPGQGLEWMGWISTYQGNTNYAQKFQGRVTMTTDTSTTTGYMELRRLRSDDTAVYYCARDYTRGAWFGESLIGGFDNWGQGTLVTVSS

SEQ ID NO: 230 - protein, 518 aa, synthetic construct
  REGION 1..518: note = Synthetic sequence SARS-CoV-2 S309-scFv-(VH-VL)-(VH-VL) v1.1
QVQLVQSGAEVKKPGASVKVSCKASGYPFTSYGISWVRQAPGQGLEWMGWISTYQGNTNYAQKFQGRVTMTTDTSTTTGYMELRRLRSDDTAVYYCARDYTRGAWFGESLIGGFDNWGQGTLVTVSSGGGGSGGGGSGGGGSEIVLTQSPGTLSLSPGERATLSCRASQTVSSTSLAWYQQKPGQAPRLLIYGASSRATGIPDRFSGSGSGTDFTLTISRLEPEDFAVYYCQQHDTSLTFGGGTKVEIKGGGGSGGGGSGGGGSGGGGSQVQLVQSGAEVKKPGASVKVSCKASGYPFTSYGISWVRQAPGQGLEWMGWISTYQGNTNYAQKFQGRVTMTTDTSTTTGYMELRRLRSDDTAVYYCARDYTRGAWFGESLIGGFDNWGQGTLVTVSSGGGGSGGGGSGGGGSEIVLTQSPGTLSLSPGERATLSCRASQTVSSTSLAWYQQKPGQAPRLLIYGASSRATGIPDRFSGSGSGTDFTLTISRLEPEDFAVYYCQQHDTSLTFGGGTKVEIK

SEQ ID NO: 231 - protein, 518 aa, synthetic construct
  REGION 1..518: note = Synthetic sequence SARS-CoV-2 S309-scFv-(VH-VL)-(VL-VH) v1.1
QVQLVQSGAEVKKPGASVKVSCKASGYPFTSYGISWVRQAPGQGLEWMGWISTYQGNTNYAQKFQGRVTMTTDTSTTTGYMELRRLRSDDTAVYYCARDYTRGAWFGESLIGGFDNWGQGTLVTVSSGGGGSGGGGSGGGGSEIVLTQSPGTLSLSPGERATLSCRASQTVSSTSLAWYQQKPGQAPRLLIYGASSRATGIPDRFSGSGSGTDFTLTISRLEPEDFAVYYCQQHDTSLTFGGGTKVEIKGGGGSGGGGSGGGGSGGGGSEIVLTQSPGTLSLSPGERATLSCRASQTVSSTSLAWYQQKPGQAPRLLIYGASSRATGIPDRFSGSGSGTDFTLTISRLEPEDFAVYYCQQHDTSLTFGGGTKVEIKGGGGSGGGGSGGGGSQVQLVQSGAEVKKPGASVKVSCKASGYPFTSYGISWVRQAPGQGLEWMGWISTYQGNTNYAQKFQGRVTMTTDTSTTTGYMELRRLRSDDTAVYYCARDYTRGAWFGESLIGGFDNWGQGTLVTVSS

SEQ ID NO: 232 - protein, 518 aa, synthetic construct
  REGION 1..518: note = Synthetic sequence SARS-CoV-2 S309-scFv-(VH-VL)-(VL-VH) v1.1
EIVLTQSPGTLSLSPGERATLSCRASQTVSSTSLAWYQQKPGQAPRLLIYGASSRATGIPDRFSGSGSGTDFTLTISRLEPEDFAVYYCQQHDTSLTFGGGTKVEIKGGGGSGGGGSGGGGSQVQLVQSGAEVKKPGASVKVSCKASGYPFTSYGISWVRQAPGQGLEWMGWISTYQGNTNYAQKFQGRVTMTTDTSTTTGYMELRRLRSDDTAVYYCARDYTRGAWFGESLIGGFDNWGQGTLVTVSSGGGGSGGGGSGGGGSGGGGSQVQLVQSGAEVKKPGASVKVSCKASGYPFTSYGISWVRQAPGQGLEWMGWISTYQGNTNYAQKFQGRVTMTTDTSTTTGYMELRRLRSDDTAVYYCARDYTRGAWFGESLIGGFDNWGQGTLVTVSSGGGGSGGGGSGGGGSEIVLTQSPGTLSLSPGERATLSCRASQTVSSTSLAWYQQKPGQAPRLLIYGASSRATGIPDRFSGSGSGTDFTLTISRLEPEDFAVYYCQQHDTSLTFGGGTKVEIK

SEQ ID NO: 233 - protein, 518 aa, synthetic construct
  REGION 1..518: note = Synthetic sequence SARS-CoV-2 S309-scFv-(VL-VH)-(VL-VH) v1.1
EIVLTQSPGTLSLSPGERATLSCRASQTVSSTSLAWYQQKPGQAPRLLIYGASSRATGIPDRFSGSGSGTDFTLTISRLEPEDFAVYYCQQHDTSLTFGGGTKVEIKGGGGSGGGGSGGGGSQVQLVQSGAEVKKPGASVKVSCKASGYPFTSYGISWVRQAPGQGLEWMGWISTYQGNTNYAQKFQGRVTMTTDTSTTTGYMELRRLRSDDTAVYYCARDYTRGAWFGESLIGGFDNWGQGTLVTVSSGGGGSGGGGSGGGGSGGGGSEIVLTQSPGTLSLSPGERATLSCRASQTVSSTSLAWYQQKPGQAPRLLIYGASSRATGIPDRFSGSGSGTDFTLTISRLEPEDFAVYYCQQHDTSLTFGGGTKVEIKGGGGSGGGGSGGGGSQVQLVQSGAEVKKPGASVKVSCKASGYPFTSYGISWVRQAPGQGLEWMGWISTYQGNTNYAQKFQGRVTMTTDTSTTTGYMELRRLRSDDTAVYYCARDYTRGAWFGESLIGGFDNWGQGTLVTVSS

SEQ ID NO: 234 - protein, 114 aa, synthetic construct
  REGION 1..114: note = Synthetic sequence SARS-CoV-2 S300-v14 mAb VL (VK)
DIVMTQSPDSLAVSLGERATINCKSSQSVLYSSNNKNYLAWYQQKPGQPPKLLISWASTRESGVPDRFSGSGSGTDFTLTISSLQAEDVAVYYCQQYYSAPGITFGQGTRLEIK

SEQ ID NO: 235 - protein, 12 aa, synthetic construct
  REGION 1..12: note = Synthetic sequence SARS-CoV-2 S300-v14 mAb CDRL1
QSVLYSSNNKNY

SEQ ID NO: 236 - skipped

SEQ ID NO: 237 - protein, 10 aa, synthetic construct
  REGION 1..10: note = Synthetic sequence SARS-CoV-2 S300-v14 mAb CDRL3
QQYYSAPGIT

SEQ ID NO: 238 - DNA, 343 bp, synthetic construct
  misc_feature 1..343: note = Synthetic sequence SARS-CoV2 S300-v14 mAb VL (VK)
  source 1..343: mol_type = other DNA
gacatcgtgatgacccagtctccagactcactggctgtgtctctgggcgagagggccaccatcaactgtaagtccagccagagtgttttatacagctccaacaataagaactacttagcttggtaccagcagaaaccaggacagcctcctaagctgctcatttcctgggcttctacccgggaatccggggtccctgaccgattcagtggcagcgggtctgggacagatttcactctcaccatcagcagcctgcaggctgaagatgtggcagtttattactgtcaacaatattatagtgctcccgggatcaccttcggccaggggacacgactggagattaaac

SEQ ID NO: 239 - protein, 129 aa, synthetic construct
  REGION 1..129: note = Synthetic sequence SARS-CoV2 S307 mAb VH
QVQLQESGPGLVKPSETLSLTCTVSGGSVTSGSYYWSWIRQPPGKGLEWIGYMYYSGSTNYNPSLKSRVTISVDTSKNQFSLKLSSVTAADTAVYYCARAGCTGITCLRYDYYYGLDVWGQGTTVTVSS

SEQ ID NO: 240 - protein, 10 aa, synthetic construct
  REGION 1..10: note = Synthetic sequence SARS-CoV2 S307 mAb CDRH1
GGSVTSGSYY

SEQ ID NO: 241 - protein, 7 aa, synthetic construct
  REGION 1..7: note = Synthetic sequence SARS-CoV2 S307 mAb CDRH2
MYYSGST

SEQ ID NO: 242 - protein, 21 aa, synthetic construct
  REGION 1..21: note = Synthetic sequence SARS-CoV2 S307 mAb CDRH3
ARAGCTGITCLRYDYYYGLDV

SEQ ID NO: 243 - protein, 108 aa, synthetic construct
  REGION 1..108: note = Synthetic sequence SARS-CoV2 S307 mAb VL(VK)
EIVLTQSPGTLSLSPGKRATLSCRASQSVSSSYLAWYQQRPGQAPRLLIYGASSRAAGIPDRFSGSGSGTDFTLTISRLEPEDFAVYYCQQYGSSSWTFGQGTKVEIK

SEQ ID NO: 244 - protein, 7 aa, synthetic construct
  REGION 1..7: note = Synthetic sequence SARS-CoV2 S307 mAb CDRL1
QSVSSSY

SEQ ID NO: 245 - skipped

SEQ ID NO: 246 - protein, 9 aa, synthetic construct
  REGION 1..9: note = Synthetic sequence SARS-CoV2 S307 mAb CDRL3
QQYGSSSWT

SEQ ID NO: 247 - DNA, 387 bp, synthetic construct
  misc_feature 1..387: note = Synthetic sequence SARS-CoV2 S307 mAb VH
  source 1..387: mol_type = other DNA
caggtgcagctgcaggagtcgggcccaggactggtgaagccttcggagaccctgtccctcacctgcactgtctctggtggctccgtcaccagtggtagttactactggagctggatccggcagcccccagggaagggactggagtggattgggtatatgtattacagtgggagcaccaattacaacccctccctcaagagtcgagtcaccatatcagtagacacgtccaagaaccagttctccctgaagctgagctctgtgaccgctgcggacacggccgtgtattactgtgcgagggcaggttgtactggtatcacctgcttacgttacgactactactacggtctggacgtctggggccaagggaccacggtcaccgtctcctca

SEQ ID NO: 248 - DNA, 325 bp, synthetic construct
  misc_feature 1..325: note = Synthetic sequence SARS-CoV2 S307 mAb VL(VK)
  source 1..325: mol_type = other DNA
gaaattgtgttgacgcagtctccaggcaccctgtctttgtctccagggaaaagagccaccctctcctgcagggccagtcagagtgttagcagcagctacttagcctggtaccagcagagacctggccaggctcccaggctcctcatctatggtgcatccagcagggccgctggcatcccagacaggttcagtggcagtgggtctgggacagacttcactctcaccatcagcagactggagcctgaagattttgcagtgtattactgtcagcagtatggtagctcatcgtggacgttcggccaagggaccaaggtggaaatcaaac

SEQ ID NO: 249 - DNA, 381 bp, synthetic construct
  misc_feature 1..381: note = Synthetic sequence SARS-CoV-2 S309-v1 mAb VH
  source 1..381: mol_type = other DNA
caggttcagctggtgcagtctggagctgaggtgaagaagcctggggcctcagtgaaggtctcctgcaaggcttctggttacccctttaccagttatggtatcagctgggtgcgacaggcccctggacaagggcttgagtggatgggatggatcagcacttacaatggtaacacaaattatgcacagaagttccagggcagagtcaccatgaccacagacacatccacgaccacaggctacatggagctgaggaggctgagatctgacgacacggccgtgtattactgtgcgagagattatactcgtggtgcttggttcggggagtcattgatagggggctttgacaactggggccagggaaccctggtcaccgtctcctca

SEQ ID NO: 250 - DNA, 322 bp, synthetic construct
  misc_feature 1..322: note = Synthetic sequence SAES-CoV-2 S309-v13 mAb VL(VK)
  source 1..322: mol_type = other DNA
gaaattgtgttgacgcagtctccaggcaccctgtctttgtctccaggggaaagagccaccctctcctgcagggccagtcagactgttagcagcacctccttagcctggtaccagcagaaacctggccaggctcccaggctcctcatctatggtgcatccagcagggccactggcatcccagacaggttcagcggcagtgggtctgggacagacttcactctcaccatcagcagactggagcctgaagattttgcagtgtattactgtcagcagcatgatacctcactcactttcggcggagggaccaaggtggagatcaaac

SEQ ID NO: 251 - DNA, 767 bp, synthetic construct
  misc_feature 1..767: note = Synthetic sequence CMV promoter
  source 1..767: mol_type = other DNA
gacattgattattgactagttattaatagtaatcaattacggggtcattagttcatagcccatatatggagttccgcgttacataacttacggtaaatggcccgcctggctgaccgcccaacgacccccgcccatgacgtcaataatgacgtatgttcccatagtaacgccaatagggactttccattgacgtcaatgggtggagtatttacggtaaactgcccacttggcagtacatcaagtgtatcatatgccaagtacgccccctattgacgtcaatgacggtaaatggcccgcctggcattatgcccagtacatgaccttatgggactttcctacttggcagtacatctacgtattagtcatcgctattaccatggtgatgcggttttggcagtacatcaatgggcgtggatagcggtttgactcacggggatttccaagtctccaccccattgacgtcaatgggagtttgttttggcaccaaaatcaacgggactttccaaaatgtcgtaacaactccgccccattgacgcaaatgggcggtaggcgtgtacggtgggaggtctatataagcagagctcgtttagtgaaccgtcagatcgcctggagacgccatccacgctgttttgacctccatagaagacaccgggaccgatccagcctccgcggccgggaacggtgcattggaacgcggattccccgtgccaagagtgacgtaagtaccgcctatagagtctataggcccacccccttggcttcgttag

SEQ ID NO: 252 - DNA, 50 bp, synthetic construct
  misc_feature 1..50: note = Signal peptide
  source 1..50: mol_type = other DNA
atgggatggtcatgtatcatcctttttctagtagcaactgcaaccggtgt

SEQ ID NO: 253 - DNA, 135 bp, synthetic construct
  misc_feature 1..135: note = Poly-adenylation signal sequence
  source 1..135: mol_type = other DNA
aacttgtttattgcagcttataatggttacaaataaagcaatagcatcacaaatttcacaaataaagcatttttttcactgcattctagttgtggtttgtccaaactcatcaatgtatcttatcatgtctggatc

SEQ ID NO: 254 - DNA, 323 bp, synthetic construct
  misc_feature 1..323: note = Synthetic sequence SARS-CoV-2 Light Chain IgKC*01
  source 1..323: mol_type = other DNA
gtacggtggctgcaccatctgtcttcatcttcccgccatctgatgagcagttgaaatctggaactgcctctgttgtgtgcctgctgaataacttctatcccagagaggccaaagtacagtggaaggtggataacgccctccaatcgggtaactcccaggagagtgtcacagagcaggacagcaaggacagcacctacagcctcagcagcaccctgacgctgagcaaagcagactacgagaaacacaaagtctacgcctgcgaagtcacccatcagggcctgagctcgcccgtcacaaagagcttcaacaggggagagtgttag

SEQ ID NO: 255 - DNA, 993 bp, synthetic construct
  misc_feature 1..993: note = Synthetic sequence SARS-CoV-2 CH1-CH3 G1m17; IgG1*01
  source 1..993: mol_type = other DNA
gcgtcgaccaagggcccatcggtcttccccctggcaccctcctccaagagcacctctgggggcacagcggccctgggctgcctggtcaaggactacttccccgaacctgtgacggtctcgtggaactcaggcgccctgaccagcggcgtgcacaccttcccggctgtcctacagtcctcaggactctactccctcagcagcgtggtgaccgtgccctccagcagcttgggcacccagacctacatctgcaacgtgaatcacaagcccagcaacaccaaggtggacaagagagttgagcccaaatcttgtgacaaaactcacacatgcccaccgtgcccagcacctgaactcctggggggaccgtcagtcttcctcttccccccaaaacccaaggacaccctcatgatctcccggacccctgaggtcacatgcgtggtggtggacgtgagccacgaagaccctgaggtcaagttcaactggtacgtggacggcgtggaggtgcataatgccaagacaaagccgcgggaggagcagtacaacagcacgtaccgtgtggtcagcgtcctcaccgtcctgcaccaggactggctgaatggcaaggagtacaagtgcaaggtctccaacaaagccctcccagcccccatcgagaaaaccatctccaaagccaaagggcagccccgagaaccacaggtgtacaccctgcccccatcccgggaggagatgaccaagaaccaggtcagcctgacctgcctggtcaaaggcttctatcccagcgacatcgccgtggagtgggagagcaatgggcagccggagaacaactacaagaccacgcctcccgtgctggactccgacggctccttcttcctctatagcaagctcaccgtggacaagagcaggtggcagcaggggaacgtcttctcatgctccgtgatgcatgaggctctgcacaaccactacacgcagaagagcctctccctgtccccgggtaaatga

SEQ ID NO: 256 - protein, 16 aa, synthetic construct
  REGION 1..16: note = Signal peptide
MGWSCIILFLVATATG

SEQ ID NO: 257 - DNA, 1431 bp, synthetic construct
  misc_feature 1..1431: note = Synthetic sequence SARS-CoV-2 S309-v1.1 mAb CH1-CH3 G1m17; IgGHG1*01 LS; GAALIE; signal peptide (nt-CO)
  source 1..1431: mol_type = other DNA
atgggctggtcctgtatcatcctgttcctggtcgccacagccaccggagtgcacagccaagtgcagctggtccagagcggcgccgaggtgaagaagcccggcgctagcgtgaaggtgtcctgtaaagccagcggatatccttttaccagctacggcatctcctgggtgcggcaggcccctggccagggcctggaatggatgggctggatcagcacctaccagggaaataccaactacgcccagaagttccagggaagagtgacaatgaccacagatacatctacaaccaccggctacatggaactgaggcggctgagaagcgacgacaccgccgtgtactactgcgccagagattacaccagaggcgcttggttcggcgagagcctgatcggcggcttcgacaactggggccagggaaccctggtgacagtgtctagcgcttctaccaaaggcccttctgtctttcctctggccccttctagcaagtctacaagcggaggcaccgccgccctgggctgcctggtgaaggactacttccccgagcccgtgaccgtgagctggaatagcggcgccctgacaagcggcgtgcacaccttcccagctgtgctgcagagcagcggcctgtatagcctgagcagcgtggtcaccgtgcccagcagcagcctgggaacacagacctacatctgcaacgtgaaccacaagccttctaataccaaggtggataagaaggtggaacctaagagctgcgacaaaacacacacatgccctccatgtcctgctccagagctgctggccggccccagcgtttttctgttcccccccaaacctaaagacaccctgatgatcagcagaacccctgaggtgacctgtgtggtggtggacgtgtcccacgaagatcctgaggtgaagttcaactggtacgtggatggagtggaagtgcacaacgccaagaccaaacctagagaagagcagtacaacagcacatatagagtcgtgtccgtgcttacagtgctgcaccaggactggctgaatggaaaggaatacaagtgcaaggtgtccaacaaggccctgcctctgcctgaggagaagacaatctctaaagccaagggccaacctcgggaacctcaggtgtacacactgccccccagccgggacgagctgaccaagaaccaggtgtccctgacctgcctggtcaagggcttctacccctctgatatcgccgtggaatgggagagcaacggccaacctgagaacaactacaagaccacccctccagtgctggacagcgacggcagcttcttcctgtacagcaagctgaccgttgacaagtccagatggcagcagggcaacgtgttcagctgtagcgtcctgcacgaggccctgcattctcactacacccagaagagcctgtccctcagccctggcaagtga

SEQ ID NO: 258 - DNA, 1374 bp, synthetic construct
  misc_feature 1..1374: note = Synthetic sequence SARS-CoV-2 S309-v1.1 mAb CH1-CH3 G1m17; IgGHG1*01 LS; GAALIE; (nt-CO)
  source 1..1374: mol_type = other DNA
caagtgcagctggtccagagcggcgccgaggtgaagaagcccggcgctagcgtgaaggtgtcctgtaaagccagcggatatccttttaccagctacggcatctcctgggtgcggcaggcccctggccagggcctggaatggatgggctggatcagcacctaccagggaaataccaactacgcccagaagttccagggaagagtgacaatgaccacagatacatctacaaccaccggctacatggaactgaggcggctgagaagcgacgacaccgccgtgtactactgcgccagagattacaccagaggcgcttggttcggcgagagcctgatcggcggcttcgacaactggggccagggaaccctggtgacagtgtctagcgcttctaccaaaggcccttctgtctttcctctggccccttctagcaagtctacaagcggaggcaccgccgccctgggctgcctggtgaaggactacttccccgagcccgtgaccgtgagctggaatagcggcgccctgacaagcggcgtgcacaccttcccagctgtgctgcagagcagcggcctgtatagcctgagcagcgtggtcaccgtgcccagcagcagcctgggaacacagacctacatctgcaacgtgaaccacaagccttctaataccaaggtggataagaaggtggaacctaagagctgcgacaaaacacacacatgccctccatgtcctgctccagagctgctggccggccccagcgtttttctgttcccccccaaacctaaagacaccctgatgatcagcagaacccctgaggtgacctgtgtggtggtggacgtgtcccacgaagatcctgaggtgaagttcaactggtacgtggatggagtggaagtgcacaacgccaagaccaaacctagagaagagcagtacaacagcacatatagagtcgtgtccgtgcttacagtgctgcaccaggactggctgaatggaaaggaatacaagtgcaaggtgtccaacaaggccctgcctctgcctgaggagaagacaatctctaaagccaagggccaacctcgggaacctcaggtgtacacactgccccccagccgggacgagctgaccaagaaccaggtgtccctgacctgcctggtcaagggcttctacccctctgatatcgccgtggaatgggagagcaacggccaacctgagaacaactacaagaccacccctccagtgctggacagcgacggcagcttcttcctgtacagcaagctgaccgttgacaagtccagatggcagcagggcaacgtgttcagctgtagcgtcctgcacgaggccctgcattctcactacacccagaagagcctgtccctcagccctggcaagtga

SEQ ID NO: 259 - DNA, 1431 bp, synthetic construct
  misc_feature 1..1431: note = Synthetic sequence SARS-CoV-2 S309-v1.1 mAb CH1-CH3 G1m17; IgGHG1*01 LS; signal peptide (nt-CO)
  source 1..1431: mol_type = other DNA
atgggctggtcctgtatcatcctgttcctggtcgccacagccaccggagtgcacagccaagtgcagctggtccagagcggcgccgaggtgaagaagcccggcgctagcgtgaaggtgtcctgtaaagccagcggatatccttttaccagctacggcatctcctgggtgcggcaggcccctggccagggcctggaatggatgggctggatcagcacctaccagggaaataccaactacgcccagaagttccagggaagagtgacaatgaccacagatacatctacaaccaccggctacatggaactgaggcggctgagaagcgacgacaccgccgtgtactactgcgccagagattacaccagaggcgcttggttcggcgagagcctgatcggcggcttcgacaactggggccagggaaccctggtgacagtgtctagcgcttctaccaaaggcccttctgtctttcctctggccccttctagcaagtctacaagcggaggcaccgccgccctgggctgcctggtgaaggactacttccccgagcccgtgaccgtgagctggaatagcggcgccctgacaagcggcgtgcacaccttcccagctgtgctgcagagcagcggcctgtatagcctgagcagcgtggtcaccgtgcccagcagcagcctgggaacacagacctacatctgcaacgtgaaccacaagccttctaataccaaggtggataagaaggtggaacctaagagctgcgacaaaacacacacatgccctccatgtcctgctccagagctgctgggcggccccagcgtttttctgttcccccccaaacctaaagacaccctgatgatcagcagaacccctgaggtgacctgtgtggtggtggacgtgtcccacgaagatcctgaggtgaagttcaactggtacgtggatggagtggaagtgcacaacgccaagaccaaacctagagaagagcagtacaacagcacatatagagtcgtgtccgtgcttacagtgctgcaccaggactggctgaatggaaaggaatacaagtgcaaggtgtccaacaaggccctgcctgcccctatcgagaagacaatctctaaagccaagggccaacctcgggaacctcaggtgtacacactgccccccagccgggacgagctgaccaagaaccaggtgtccctgacctgcctggtcaagggcttctacccctctgatatcgccgtggaatgggagagcaacggccaacctgagaacaactacaagaccacccctccagtgctggacagcgacggcagcttcttcctgtacagcaagctgaccgttgacaagtccagatggcagcagggcaacgtgttcagctgtagcgtcctgcacgaggccctgcattctcactacacccagaagagcctgtccctcagccctggcaagtga

SEQ ID NO: 260 - DNA, 1374 bp, synthetic construct
  misc_feature 1..1374: note = Synthetic sequence SARS-CoV-2 S309-v1.1 mAb CH1-CH3 G1m17; IgGHG1*01 LS (nt-CO)
  source 1..1374: mol_type = other DNA
caagtgcagctggtccagagcggcgccgaggtgaagaagcccggcgctagcgtgaaggtgtcctgtaaagccagcggatatccttttaccagctacggcatctcctgggtgcggcaggcccctggccagggcctggaatggatgggctggatcagcacctaccagggaaataccaactacgcccagaagttccagggaagagtgacaatgaccacagatacatctacaaccaccggctacatggaactgaggcggctgagaagcgacgacaccgccgtgtactactgcgccagagattacaccagaggcgcttggttcggcgagagcctgatcggcggcttcgacaactggggccagggaaccctggtgacagtgtctagcgcttctaccaaaggcccttctgtctttcctctggccccttctagcaagtctacaagcggaggcaccgccgccctgggctgcctggtgaaggactacttccccgagcccgtgaccgtgagctggaatagcggcgccctgacaagcggcgtgcacaccttcccagctgtgctgcagagcagcggcctgtatagcctgagcagcgtggtcaccgtgcccagcagcagcctgggaacacagacctacatctgcaacgtgaaccacaagccttctaataccaaggtggataagaaggtggaacctaagagctgcgacaaaacacacacatgccctccatgtcctgctccagagctgctgggcggccccagcgtttttctgttcccccccaaacctaaagacaccctgatgatcagcagaacccctgaggtgacctgtgtggtggtggacgtgtcccacgaagatcctgaggtgaagttcaactggtacgtggatggagtggaagtgcacaacgccaagaccaaacctagagaagagcagtacaacagcacatatagagtcgtgtccgtgcttacagtgctgcaccaggactggctgaatggaaaggaatacaagtgcaaggtgtccaacaaggccctgcctgcccctatcgagaagacaatctctaaagccaagggccaacctcgggaacctcaggtgtacacactgccccccagccgggacgagctgaccaagaaccaggtgtccctgacctgcctggtcaagggcttctacccctctgatatcgccgtggaatgggagagcaacggccaacctgagaacaactacaagaccacccctccagtgctggacagcgacggcagcttcttcctgtacagcaagctgaccgttgacaagtccagatggcagcagggcaacgtgttcagctgtagcgtcctgcacgaggccctgcattctcactacacccagaagagcctgtccctcagccctggcaagtga

SEQ ID NO: 261 - DNA, 701 bp, synthetic construct
  misc_feature 1..701: note = Synthetic sequence S309-v13 Light chain k1m3; IgKC*01; signal peptide (nt-CO)
  source 1..701: mol_type = other DNA
tgggctggtcctgcatcatcctgttcctggtggccacagccaccggcgtgcacagcgagatcgtcctgacacagagccccggcacactgagcctctccccaggcgagcgggctacactgtcttgtagagcttctcagaccgtgtccagcaccagcctggcctggtatcagcagaaacctggccaggcccctagactgctgatctacggcgccagcagcagagccaccggcatccctgatagattcagcggcagcggatctggaaccgacttcaccctgaccatcagccggctggaacccgaggactttgccgtgtactactgccagcaacacgacaccagcctgaccttcggcggcggaacaaaggtggaaatcaagagaaccgtggccgcccctagcgtgttcatcttcccccccagcgacgagcagctgaagagcggtacagcttctgtggtgtgcctgctgaacaacttctacccgcgggaagccaaggtgcagtggaaggtggacaacgccctgcagagcggcaacagccaggagagcgtgacagagcaggacagcaaggacagcacctacagcctgagcagcaccctgaccctgagcaaggccgactacgagaagcacaaggtgtacgcctgtgaagtgacccaccagggcctgtctagccctgtgaccaagtcttttaacagaggcgagtgctga

SEQ ID NO: 262 - DNA, 645 bp, synthetic construct
  misc_feature 1..645: note = Synthetic sequence S309-v13 Light chain k1m3; IgKC*01; (nt-CO)
  source 1..645: mol_type = other DNA
gagatcgtcctgacacagagccccggcacactgagcctctccccaggcgagcgggctacactgtcttgtagagcttctcagaccgtgtccagcaccagcctggcctggtatcagcagaaacctggccaggcccctagactgctgatctacggcgccagcagcagagccaccggcatccctgatagattcagcggcagcggatctggaaccgacttcaccctgaccatcagccggctggaacccgaggactttgccgtgtactactgccagcaacacgacaccagcctgaccttcggcggcggaacaaaggtggaaatcaagagaaccgtggccgcccctagcgtgttcatcttcccccccagcgacgagcagctgaagagcggtacagcttctgtggtgtgcctgctgaacaacttctacccgcgggaagccaaggtgcagtggaaggtggacaacgccctgcagagcggcaacagccaggagagcgtgacagagcaggacagcaaggacagcacctacagcctgagcagcaccctgaccctgagcaaggccgactacgagaagcacaaggtgtacgcctgtgaagtgacccaccagggcctgtctagccctgtgaccaagtcttttaacagaggcgagtgctga

SEQ ID NO: 263 - DNA, 57 bp, synthetic construct
  misc_feature 1..57: note = Signal peptide
  source 1..57: mol_type = other DNA
atgggctggtcctgcatcatcctgttcctggtggccacagccaccggcgtgcacagc

SEQ ID NO: 264 - protein, 19 aa, synthetic construct
  REGION 1..19: note = Signal peptide
MGWSCIILFLVATATGVHS

SEQ ID NO: 265 - protein, 329 aa, synthetic construct
  REGION 1..329: note = Synthetic sequence SARS-CoV-2 CH1-CH3 G1m17; IgG1*01 LS no C-term Lys
ASTKGPSVFPLAPSSKSTSGGTAALGCLVKDYFPEPVTVSWNSGALTSGVHTFPAVLQSSGLYSLSSVVTVPSSSLGTQTYICNVNHKPSNTKVDKKVEPKSCDKTHTCPPCPAPELLGGPSVFLFPPKPKDTLMISRTPEVTCVVVDVSHEDPEVKFNWYVDGVEVHNAKTKPREEQYNSTYRVVSVLTVLHQDWLNGKEYKCKVSNKALPAPIEKTISKAKGQPREPQVYTLPPSRDELTKNQVSLTCLVKGFYPSDIAVEWESNGQPENNYKTTPPVLDSDGSFFLYSKLTVDKSRWQQGNVFSCSVLHEALHSHYTQKSLSLSPG

SEQ ID NO: 266 - protein, 329 aa, synthetic construct
  REGION 1..329: note = Synthetic sequence SARS-CoV-2 CH1-CH3 G1m17; IgG1*01 LS GAALIE no C-term Lys
ASTKGPSVFPLAPSSKSTSGGTAALGCLVKDYFPEPVTVSWNSGALTSGVHTFPAVLQSSGLYSLSSVVTVPSSSLGTQTYICNVNHKPSNTKVDKKVEPKSCDKTHTCPPCPAPELLAGPSVFLFPPKPKDTLMISRTPEVTCVVVDVSHEDPEVKFNWYVDGVEVHNAKTKPREEQYNSTYRVVSVLTVLHQDWLNGKEYKCKVSNKALPLPEEKTISKAKGQPREPQVYTLPPSRDELTKNQVSLTCLVKGFYPSDIAVEWESNGQPENNYKTTPPVLDSDGSFFLYSKLTVDKSRWQQGNVFSCSVLHEALHSHYTQKSLSLSPG

SEQ ID NO: 267 - protein, 127 aa, synthetic construct
  REGION 1..127: note = SARS-CoV-2 S309 VH consensus sequence
  VARIANT 50: note = Xaa = W, F, or Y
  VARIANT 55: note = Xaa = N, Q, L, or T
  VARIANT 56: note = Xaa = G, S, A, or Q
  VARIANT 105: note = Xaa = W, F, or Y
QVQLVQSGAEVKKPGASVKVSCKASGYPFTSYGISWVRQAPGQGLEWMGXISTYXXNTNYAQKFQGRVTMTTDTSTTTGYMELRRLRSDDTAVYYCARDYTRGAXFGESLIGGFDNWGQGTLVTVSS